European Patent Specification EP 3 820 884 B1, published September 3, 2025. Title: METHOD FOR RESCUING AND PRODUCING A VIRUS IN AVIAN CELLS. Applicant: Valneva SE. The sequence listing filed with the application follows.

SEQUENCE LISTING (136 sequences)

SEQ ID NO: 1 - protein, 6 aa, Newcastle disease virus
GRQGRL

SEQ ID NO: 2 - protein, 6 aa, Newcastle disease virus
RRQKRL

SEQ ID NO: 3 - protein, 6 aa, Newcastle disease virus
RRRRRL

SEQ ID NO: 4 - protein, 6 aa, Newcastle disease virus
RRQRRF

SEQ ID NO: 5 - protein, 6 aa, Newcastle disease virus
KKRKRL

SEQ ID NO: 6 - DNA, 18 bp, T7 bacteriophage
taatacgactactatagg

SEQ ID NO: 7 - DNA, 24 bp, T7 bacteriophage
taaacgggtcttgaggggtttttt

SEQ ID NO: 8 - DNA, 106 bp, Hepatitis D virus
cccagccgtaccgttctccacctcctcgcggtccgacctgggcatccgaaggaggacgcacgtccactcggatggctaagggagtagcataaccccttggggcctc

SEQ ID NO: 9 - DNA, 62 bp, Artificial Sequence
  Artificial sequence
aattcttttcgccggcgtggccggcctttaattaatcctgcaggtcttaagtgcgatcgcta

SEQ ID NO: 10 - DNA, 62 bp, Artificial Sequence
  Artificial sequence
agcttagcgatcgcacttaagacctgcaggattaattaaaggccggccacgccggcgaaaag

SEQ ID NO: 11 - DNA, 3242 bp, Artificial Sequence
  Artificial sequence
cgccggcgtaatacgactcactatagggaccaaacagagaatccgtgagttacgataaaaggcgaaggagcaattgaagtcgcacgggtagaaggtgtgaatctcgagtgcgagcccgaagcacaaactcgagaaagccttctgccaacatgtcttccgtatttgatgagtacgaacagctcctcgcggctcagactcgccccaatggagctcatggagggggagaaaaagggagtaccttaaaagtagacgtcccggtattcactcttaacagtgatgacccagaagatagatggagctttgtggtattctgcctccggattgctgttagcgaagatgccaacaaaccactcaggcaaggtgctctcatatctcttttatgctcccactcacaggtaatgaggaaccatgttgccattgcagggaaacagaatgaagccacattggccgtgcttgagattgatggctttgccaacggcacgccccagttcaacaataggagtggagtgtctgaagagagagcacagagatttgcgatgatagcaggatctctccctcgggcatgcagcaacggaaccccgttcgtcacagccggggcagaagatgatgcaccagaagacatcaccgataccctggagaggatcctctctatccaggctcaagtatgggtcacagtagcaaaagccatgactgcgtatgagactgcagatgagtcggaaacaaggcgaatcaataagtatatgcagcaaggcagggtccaaaagaaatacatcctctaccccgtatgcaggagcacaatccaactcacgatcagacagtctcttgcagtccgcatctttttggttagcgagctcaagagaggccgcaacacggcaggtggtacctctacttattataacctggtaggggacgtagactcatacatcaggaataccgggcttactgcattcttcttgacactcaagtacggaatcaacaccaagacatcagcccttgcacttagtagcctctcaggcgacatccagaagatgaagcagctcatgcgtttgtatcggatgaaaggagataatgcgccgtacatgacattacttggtgatagtgaccagatgagctttgcgcctgccgagtatgcacaactttactcctttgccatgggtatggcatcagtcctagataaaggtactgggaaataccaatttgccagggactttatgagcacatcattctggagacttggagtagagtacgctcaggctcagggaagtagcattaacgaggatatggctgccgagctaaagctaaccccagcagcaatgaagggcctggcagctgctgcccaacgggtctccgacgataccagcagcatatacatgcctactcaacaagtcggagtcctcactgggcttagcgagggggggtcccaagctctacaaggcggatcgaatagatcgcaagggcaaccagaagccggggatggggagacccaattcctggatctgatgagagcggtagcaaatagcatgagggaggcgccaaactctgcacagggcactccccaatcggggcctcccccaactcctgggccatcccaagataacgacaccgactgggggtattgatggacaaaacccagcctgcttccacaaaaacatcccaatgccctcacccgtagtcgacccctcgatttgcggctctatatgaccacaccctcaaacaaacatccccctctttcctccctccccctgctgtacaactcggcgcgccctagataccacaggcacaatgcggctcactaacaatcaaaacagagccgagggaattagaaaaaagtacgggtagaagagggatattcagagatcagggcaagtctcccgagtctctgctctctcctctacctgatagaccaggacaaacatggccacctttacagatgcagagatcgacgagctatttgagacaagtggaactgtcattgacaacataattacagcccagggtaaaccagcagagactgttggaaggagtgcaatcccacaaggcaagaccaaggtgctgagcgcagcatgggagaagcatgggagcatccagccaccggccagtcaagacaaccccgatcgacaggacagatctgacaaacaaccatccacacccgagcaaacgaccccgcatgacagcccgccggccacatccgccgaccagccccccacccaggccacagacgaagccgtcgacacacagttcaggaccggagcaagcaactctctgctgttgatgcttgacaagctcagcaataaatcgtccaatgctaaaaagggcccatggtcgagcccccaagaggggaatcaccaacgtccgactcaacagcaggggagtcaacccagtcgcggaaacagtcaggaaagaccgcagaaccaagtcaaggccgcccctggaaaccagggcacagacgtgaacacagcatatcatggacaatgggaggagtcacaactatcagctggtgcaacccctcatgctctccgatcaaggcagagccaagacaatacccttgtatctgcggatcatgtccagccacctgtagactttgtgcaagcgatgatgtctatgatggaggcgatatcacagagagtaagtaaggttgactatcagctagatcttgtcttgaaacagacatcctccatccctatgatgcggtccgaaatccaacagctgaaaacatctgttgcagtcatggaagccaacttgggaatgatgaagattctggatcccggttgtgccaacatttcatctctgagtgatctacgggcagttgcccgatctcacccggttttagtttcaggccctggagacccctctccctatgtgacacaaggaggcgaaatggcacttaataaactttcgcaaccagtgccacatccatctgaattgattaaacccgccactgcatgcgggcctgatataggagtggaaaaggacactgtccgtgcattgatcatgtcacgcccaatgcacccgagttcttcagccaagctcctaagcaagttagatgcagccgggtcgatcgaggaaatcaggaaaatcaagcgccttgctctaaatggctaattactactgccacacgtagcgggtccctgtccactcggcatcacacggaatctgcaccgagttcccccccgcagacccaaggtccaactctccaagcggcaatcctctctcgcttcctcagccccactgaatggccggcc

SEQ ID NO: 12 - DNA, 2971 bp, Artificial Sequence
  Artificial sequence
ggccggccaaccgtaattaatctagctacatttaagattaagaaaaaatacgggtagaattggagtgccccaattgtgccaagatggactcatctaggacaattgggctgtactttgattctgcccattcttctagcaacctgttagcatttccgatcgtcctacaaggcacaggagatgggaagaagcaaatcgccccgcaatataggatccagcgccttgacttgtggactgatagtaaggaggactcagtattcatcaccacctatggattcatctttcaagttgggaatgaagaagccactgtcggcatgatcgatgataaacccaagcgcgagttactttccgctgcgatgctctgcctaggaagcgtcccaaataccggagaccttattgagctggcaagggcctgtctcactatgatagtcacatgcaagaagagtgcaactaatactgagagaatggttttctcagtagtgcaggcaccccaagtgctgcaaagctgtagggttgtggcaaacaaatactcatcagtgaatgcagtcaagcacgtgaaagcgccagagaagattcccgggagtggaaccctagaatacaaggtgaactttgtctccttgactgtggtaccgaagaaggatgtctacaagatcccagctgcagtattgaaggtttctggctcgagtctgtacaatcttgcgctcaatgtcactattaatgtggaggtagacccgaggagtcctttggttaaatctttgtctaagtctgacagcggatactatgctaacctcttcttgcatattggacttatgaccaccgtagataggaaggggaagaaagtgacatttgacaagctggaaaagaaaataaggagccttgatctatctgtcgggctcagtgatgtgctcgggccttccgtgttggtaaaagcaagaggtgcacggactaagcttttggcacctttcttctctagcagtgggacagcctgctatcccatagcaaatgcttctcctcaggtggccaagatactctggagtcaaaccgcgtgcctgcggagcgttaaaatcattatccaagcaggtacccaacgcgctgtcgcagtgaccgccgaccacgaggttacctctactaagctggagaaggggcacacccttgccaaatacaatccttttaagaaataagctgcgtctctgagattgcgctccgcccactcacccagatcatcatgacacaaaaaactaatctgtcttgattatttacagttagtttacgcgtctatcaagttagaaaaaacacgggtagaagattctggatcccggttggcgccctccaggtgcaagatgggctccagaccttctaccaagaacccagcacctatgatgctgactatccgggttgcgctggtactgagttgcatctgtccggcaaactccattgatggcaggcctcttgcagctgcaggaattgtggttacaggagacaaagccgtcaacatatacacctcatcccagacaggatcaatcatagttaagctcctcccgaatctgcccaaggataaggaggcatgtgcgaaagcccccttggatgcatacaacaggacattgaccactttgctcaccccccttggtgactctatccgtaggatacaagagtctgtgactacatctggaggggggagacaggggcgccttataggcgccattattggcggtgtggctcttggggttgcaactgccgcacaaataacagcggccgcagctctgatacaagccaaacaaaatgctgccaacatcctccgacttaaagagagcattgccgcaaccaatgaggctgtgcatgaggtcactgacggattatcgcaactagcagtggcagttgggaagatgcagcagtttgttaatgaccaatttaataaaacagctcaggaattagactgcatcaaaattgcacagcaagttggtgtagagctcaacctgtacctaaccgaattgactacagtattcggaccacaaatcacttcacctgctttaaacaagctgactattcaggcactttacaatctagctggtggaaatatggattacttattgactaagttaggtgtagggaacaatcaactcagctcattaatcggtagcggcttaatcaccggtaaccctattctatacgactcacagactcaactcttgggtatacaggtaactctaccttcagtcgggaacctaaataatatgcgtgccacctacttggaaaccttatccgtaagcacaaccaggggatttgcctcggcacttgtccccaaagtggtgacacaggtcggttctgtgatagaagaacttgacacctcatactgtatagaaactgacttagatttatattgtacaagaatagtaacgttccctatgtcccctggtatttattcctgcttgagcggcaatacgtcggcctgtatgtactcaaagaccgaaggcgcacttactacaccatacatgactatcaaaggttcagtcatcgccaactgcaagatgacaacatgtagatgtgtaaaccccccgggtatcatatcgcaaaactatggagaagccgtgtctctaatagataaacaatcatgcaatgttttatccttaggcgggataactttaaggctcagtggggaattcgatgtaacttatcagaagaatatctcaatacaagattctcaagtaataataacaggcaatcttgatatctcaactgagcttgggaatgtcaacaactcgatcagtaatgctttgaataagttagaggaaagcaacagaaaactagacaaagtcaatgtcaaactgactagcacatctgctctcattacctatatcgttttgactatcatatctcttgtttttggtatacttagcctgattctagcatgctacctaatgtacaagcaaaaggcgcaacaaaagaccttattatggcttgggaataatactctaga

SEQ ID NO: 13 - DNA, 3092 bp, Artificial Sequence
  Artificial sequence
ttaattaagtgaaagttctggtagtctgtcagttcagagagttaagaaaaaactaccggttgtagatgaccaaaggacgatatacgggtagaacggtaagagaggccgcccctcaattgcgagccaggcttcacaacctccgttctaccgcttcaccgacaacagtcctcaatcatggaccgcgccgttagccaagttgcgttagagaatgatgaaagagaggcaaaaaatacatggcgcttgatattccggattgcaatcttattcttaacagtagtgaccttggctatatctgtagcctcccttttatatagcatgggggctagcacacctagcgatcttgtaggcataccgactaggatttccagggcagaagaaaagattacatctacacttggttccaatcaagatgtagtagataggatatataagcaagtggcccttgagtctccgttggcattgttaaatactgagaccacaattatgaacgcaataacatctctctcttatcagattaatggagctgcaaacaacagtgggtggggggcacctatccatgacccagattatataggggggataggcaaagaactcattgtagatgatgctagtgatgtcacatcattctatccctctgcatttcaagaacatctgaattttatcccggcgcctactacaggatcaggttgcactcgaataccctcatttgacatgagtgctacccattactgctacacccataatgtaatattgtctggatgcagagatcactcacattcatatcagtatttagcacttggtgtgctccggacatctgcaacagggagggtattcttttctactctgcgttccatcaacctggacgacacccaaaatcggaagtcttgcagtgtgagtgcaactcccctgggttgtgatatgctgtgctcgaaagtcacggagacagaggaagaagattataactcagctgtccctacgcggatggtacatgggaggttagggttcgacggccagtaccacgaaaaggacctagatgtcacaacattattcggggactgggtggccaactacccaggagtagggggtggatcttttattgacagccgcgtatggttctcagtctacggagggttaaaacccaattcacccagtgacactgtacaggaagggaaatatgtgatatacaagcgatacaatgacacatgcccagatgagcaagactaccagattcgaatggccaagtcttcgtataagcctggacggtttggtgggaaacgcatacagcaggctatcttatctatcaaggtgtcaacatccttaggcgaagacccggtactgactgtaccgcccaacacagtcacactcatgggggccgaaggcagaattctcacagtagggacatctcatttcttgtatcaacgagggtcatcatacttctctcccgcgttattatatcctatgacagtcagcaacaaaacagccactcttcatagtccttatacattcaatgccttcactcggccaggtagtatcccttgccaggcttcagcaagatgccccaactcgtgtgttactggagtctatacagatccatatcccctaatcttctatagaaaccacaccttgcgaggggtattcgggacaatgcttgatggtgtacaagcaagacttaaccctgcgtctgcagtattcgatagcacatcccgcagtcgcattactcgagtgagttcaagcagtaccaaagcagcatacacaacatcaacttgttttaaagtggtcaagactaataagacctattgtctcagcattgctgaaatatctaatactctcttcggagaattcagaatcgtcccgttactagttgagatcctcaaagatgacggggttagagaagccaggtctggctagttgagtcaattataaaggagttggaaagatggcattgtatcacctatcttctgcgacatcaagaatcaaaccgaatggccgcgcgggcccgaattccatgttgccagttgaccacaatcagccagtgctcatgcgatcagattaagccttgtcattaatctcttgattaagaaaaaatgtaagtggcaatgagatacaaggcaaaacagctcatggtaaataatacgggtaggacatggcgagctccggtcctgaaagggcagagcatcagattatcctaccagagccacacctgtcttcaccattggtcaagcacaaactactctattactggaaattaactgggctaccgcttcctgatgaatgtgacttcgaccacctcattctcagccgacaatggaaaaaaatacttgaatcggcctctcctgatactgagagaatgataaaactcggaagggcagtacaccaaactcttaaccacaattccagaataaccggagtgctccaccccaggtgtttagaacaactggctaatattgaggtcccagattcaaccaacaaatttcggaagattgagaagaagatccaaattcacaacacgagatatggagaactgttcacaaggctgtgtacgcatatagagaagaaactgctggggtcatcttggtctaacaatgtcccccggtcagaggagttcagcagcattcgtacggatccggcattctggtttcactcaaaatggtccacagccaagtttgcatggctccatataaaacagatccagaggcatctgatggtggcagctaagacaaggtctgcggccaacaaattggtgatgctaacccataaggtaggccaagtctttgtcactcctgaacttgtcgttgtgacgcatacgaatgagaacaagttcacatgtcttacccaggaacttgtattgatgtatgcagatatgatggagggcagagatatggtcaacataatatcaaccacggcggtgcatctcagaagcttatcagagaaaattgatgacattttgcggttaatagacgctctggcaaaagacttgggtaatcaagtctacgatgttgtatcactaatggagggatttgcatacggagctgtccagctactcgagccgtcaggtacatttgcaggagatttcttcgcattcaacctgcagg

SEQ ID NO: 14 - DNA, 2035 bp, Artificial Sequence
  Artificial sequence
cctgcaggagcttaaagacattctaattggcctcctccccaatgatatagcagaatccgtgactcatgcaatcgctactgtattctctggtttagaacagaatcaagcagctgagatgttgtgtctgttgcgtctgtggggtcacccactgcttgagtcccgtattgcagcaaaggcagtcaggagccaaatgtgcgcaccgaaaatggtagactttgatatgatccttcaggtactgtctttcttcaagggaacaatcatcaacgggtacagaaagaagaatgcaggtgtgtggccgcgagtcaaagtggatacaatatatgggaaggtcattgggcaactacatgcagattcagcagagatttcacacgatatcatgttgagagagtataagagtttatctgcacttgaatttgagccatgtatagaatatgaccctgtcaccaacctgagcatgttcctaaaagacaaggcaatcgcacaccccaacgataattggcttgcctcgtttaggcggaaccttctctccgaagaccagaagaaacatgtaaaagaagcaacttcgactaatcgcctcttgatagagtttttagagtcaaatgattttgatccatataaagagatggaatatctgacgacccttgagtaccttagagatgacaatgtggcagtatcatactcgctcaaggagaaggaagtgaaagttaatggacggatcttcgctaagctgacaaagaagttaaggaactgtcaggtgatggcggaagggatcctagccgatcagattgcacctttctttcagggaaatggagtcattcaggatagcatatccttgaccaagagtatgctagcgatgagtcaactgtcttttaacagcaataagaaacgtatcactgactgtaaagaaagagtatcttcaaaccgcaatcatgatccgaaaagcaagaaccgtcggagagttgcaaccttcataacaactgacctgcaaaagtactgtcttaattggagatatcagacaatcaaattgttcgctcatgccatcaatcagttgatgggcctacctcacttcttcgaatggattcacctaagactgatggacactacgatgttcgtaggagaccctttcaatcctccaagtgaccctactgactgtgacctctcaagagtccctaatgatgacatatatattgtcagtgccagagggggtatcgaaggattatgccagaagctatggacaatgatctcaattgctgcaatccaacttgctgcagctagatcgcattgtcgtgttgcctgtatggtacagggtgataatcaagtaatagcagtaacgagagaggtaagatcagacgactctccggagatggtgttgacacagttgcatcaagccagtgataatttcttcaaggaattaattcatgtcaatcatttgattggccataatttgaaggatcgtgaaaccatcaggtcagacacattcttcatatacagcaaacgaatcttcaaagatggagcaatcctcagtcaagtcctcaaaaattcatctaaattagtgctagtgtcaggtgatctcagtgaaaacaccgtaatgtcctgtgccaacattgcctctactgtagcacggctatgcgagaacgggcttcccaaagacttctgttactatttaaactatataatgagttgtgtgcagacatactttgactctgagttctccatcaccaacaattcgcaccccgatcttaatcagtcgtggattgaggacatctcttttgtgcactcatatgttctgactcctgcccaattagggggactgagtaaccttcaatactcaaggctctacactagaaatatcggtgacccggggactactgcttttgcagagatcaagcgactagaagcagtgggattactgagtcctaacattatgactaatatcttaactaggccgcctgggaatggagattgggccagtctgtgcaacgacccatactctttcaattttgagactgttgcaagcccaaatattgttcttaag

SEQ ID NO: 15 - DNA, 3975 bp, Artificial Sequence
  Artificial sequence
cttaagaaacatacgcaaagagtcctatttgaaacttgttcaaatcccttattgtctggagtgcacacagaggataatgaggcagaagagaaggcattggctgaattcttgcttaatcaagaggtgattcatccccgcgttgcgcatgccatcatggaggcaagctctgtaggtaggagaaagcaaattcaagggcttgttgacacaacaaacaccgtaattaagattgcgcttactaggaggccattaggcatcaagaggctgatgcggatagtcaattattctagcatgcatgcaatgctgtttagagacgatgttttttcctccagtagatccaaccaccccttagtctcttctaatatgtgttctctgacactggcagactatgcacggaatagaagctggtcacctttgacgggaggcaggaaaatactgggtgtatctaatcctgatacgatagaactcgtagagggtgagattcttagtgtaagcggagggtgtacaagatgtgacagcggagatgaacaatttacttggttccatcttccaagcaatatagaattgaccgatgacaccagcaagaatcctccgatgagggtaccatatctcgggtcaaagacacaggagaggagagctgcctcacttgcaaaaatagctcatatgtcgccacatgtaaaggctgccctaagggcatcatccgtgttgatctgggcttatggggataatgaagtaaattggactgctgctcttacgattgcaaaatctcggtgtaatgtaaacttagagtatcttcggttactgtcccctttacccacggctgggaatcttcaacatagactagatgatggtataactcagatgacattcacccctgcatctctctacaggtgtcaccttacattcacatatccaatgattctcaaaggctgttcactgaagaaggagtcaaagaggggaatgtggtttaccaacagagtcatgctcttgggtttatctctaatcgaatcgatctttccaatgacaacaaccaggacatatgatgagatcacactgcacctacatagtaaatttagttgctgtatcagagaagcacctgttgcggttcctttcgagctacttggggtggtaccggaactgaggacagtgacctcaaataagtttatgtatgatcctagccctgtatcggagggagactttgcgagacttgacttagctatcttcaagagttatgagcttaatctggagtcatatcccacgatagagctaatgaacattctttcaatatccagcgggaagttgattggccagtctgtggtttcttatgatgaagatacctccataaagaatgacgccataatagtgtatgacaatacccgaaattggatcagtgaagctcagaattcagatgtggtccgcctatttgaatatgcagcacttgaagtgctcctcgactgttcttaccaactctattacctgagagtaagaggcctagacaatattgtcttatatatgggtgatttatacaagaatatgccaggaattctactttccaacattgcagctacaatatctcatcccgtcattcattcaaggttacatgcagtgggcctggtcaaccatgacggatcacaccaacttgcagatacggattttatcgaaatgtctgcaaaactattagtatcttgcacccgacgtgtgatctccggcttatattcaggaaataagtatgatctgctgttcccatctgtcttagatgataacctgaatgagaagatgcttcagctgatatcccggttatgctgtctgtacacggtactctttgctacaacaagagaaatcccgaaaataagaggcttaactgcagaagagaaatgttcaatactcactgagtatttactgtcggatgctgtgaaaccattacttagccccgatcaagtgagctctatcatgtctcctaacataattacattcccagctaatctgtactacatgtctcggaagagcctcaatttgatcagggaaagggaggacagggatactatcctggcgttgttgttcccccaagagccattattagagttcccttctgtgcaagatattggtgctcgagtgaaagatccattcacccgacaacctgcggcatttttgcaagagttagatttgagtgctccagcaaggtatgacgcattcacacttagtcagattcatcctgaactcacatctccaaatccggaggaagactacttagtacgatacttgttcagagggatagggactgcatcttcctcttggtataaggcatctcatctcctttctgtacccgaggtaagatgtgcaagacacgggaactccttatacttagctgaagggagcggagccatcatgagtcttctcgaactgcatgtaccacatgaaactatctattacaatacgctcttttcaaatgagatgaaccccccgcaacgacatttcgggccgaccccaactcagtttttgaattcggttgtttataggaatctacaggcggaggtaacatgcaaagatggatttgtccaagagttccgtccattatggagagaaaatacagaggaaagtgacctgacctcagataaagcagtggggtatattacatctgcagtgccctacagatctgtatcattgctgcattgtgacattgaaattcctccagggtccaatcaaagcttactagatcaactagctatcaatttatctctgattgccatgcattctgtaagggagggcggggtagtaatcatcaaagtgttgtatgcaatgggatactactttcatctactcatgaacttgtttgctccgtgttccacaaaaggatatattctctctaatggttatgcatgtcgaggagatatggagtgttacctggtatttgtcatgggttacctgggcgggcctacatttgtacatgaggtggtgaggatggcaaaaactctggtgcagcggcacggtacgctcttgtctaaatcagatgagatcacactgaccaggttattcacctcacagcggcagcgtgtgacagacatcctatccagtcctttaccaagattaataaagtacttgaggaagaatattgacactgcgctgattgaagccgggggacagcccgtccgtccattctgtgcggagagtctggtgagcacgctagcgaacataactcagataacccagattatcgctagtcacattgacacagttatccggtctgtgatatatatggaagctgagggtgatctcgctgacacagtatttctatttaccccttacaatctctctactgacgggaaaaagaggacatcacttatacagtgcacgagacagatcctagaggttacaatactaggtcttagagtcgaaaatctcaataaaataggcgatataatcagcctagtgcttaaaggcatgatctccatggaggaccttatcccactaaggacatacttgaagcatagtacctgccctaaatatttgaaggctgtcctaggtattaccaaactcaaagaaatgtttacagacacttctgtattgtacttgactcgtgctcaacaaaaattctacatgaaaactataggcaatgcagtcaaaggatattacagtaactgtgactcttaacgaaaatcacatattaataggctccttttttggccaattgtattcttgttgatttaatcatattatgttagaaaaaagttgaaccctgactccttaggactcgaattcgaactcaaataaatgtcttaaaaaaaggttgcgcacaattattcttgagtgtagtctcgtcattcaccaaatctttgtttggtgggtcggcatggcatctccacctcctcgcggtccgacctgggcatccgaaggaggacgcacgtccactcggatggctaagggagtagcataaccccttggggcctctaaacgggtcttgaggggttttttggcgatcgc

SEQ ID NO: 16 - DNA, 15186 bp, Artificial Sequence
  Artificial sequence
accaaacagagaatccgtgagttacgataaaaggcgaaggagcaattgaagtcgcacgggtagaaggtgtgaatctcgagtgcgagcccgaagcacaaactcgagaaagccttctgccaacatgtcttccgtatttgatgagtacgaacagctcctcgcggctcagactcgccccaatggagctcatggagggggagaaaaagggagtaccttaaaagtagacgtcccggtattcactcttaacagtgatgacccagaagatagatggagctttgtggtattctgcctccggattgctgttagcgaagatgccaacaaaccactcaggcaaggtgctctcatatctcttttatgctcccactcacaggtaatgaggaaccatgttgccattgcagggaaacagaatgaagccacattggccgtgcttgagattgatggctttgccaacggcacgccccagttcaacaataggagtggagtgtctgaagagagagcacagagatttgcgatgatagcaggatctctccctcgggcatgcagcaacggaaccccgttcgtcacagccggggcagaagatgatgcaccagaagacatcaccgataccctggagaggatcctctctatccaggctcaagtatgggtcacagtagcaaaagccatgactgcgtatgagactgcagatgagtcggaaacaaggcgaatcaataagtatatgcagcaaggcagggtccaaaagaaatacatcctctaccccgtatgcaggagcacaatccaactcacgatcagacagtctcttgcagtccgcatctttttggttagcgagctcaagagaggccgcaacacggcaggtggtacctctacttattataacctggtaggggacgtagactcatacatcaggaataccgggcttactgcattcttcttgacactcaagtacggaatcaacaccaagacatcagcccttgcacttagtagcctctcaggcgacatccagaagatgaagcagctcatgcgtttgtatcggatgaaaggagataatgcgccgtacatgacattacttggtgatagtgaccagatgagctttgcgcctgccgagtatgcacaactttactcctttgccatgggtatggcatcagtcctagataaaggtactgggaaataccaatttgccagggactttatgagcacatcattctggagacttggagtagagtacgctcaggctcagggaagtagcattaacgaggatatggctgccgagctaaagctaaccccagcagcaatgaagggcctggcagctgctgcccaacgggtctccgacgataccagcagcatatacatgcctactcaacaagtcggagtcctcactgggcttagcgagggggggtcccaagctctacaaggcggatcgaatagatcgcaagggcaaccagaagccggggatggggagacccaattcctggatctgatgagagcggtagcaaatagcatgagggaggcgccaaactctgcacagggcactccccaatcggggcctcccccaactcctgggccatcccaagataacgacaccgactgggggtattgatggacaaaacccagcctgcttccacaaaaacatcccaatgccctcacccgtagtcgacccctcgatttgcggctctatatgaccacaccctcaaacaaacatccccctctttcctccctccccctgctgtacaactcggcgcgccctagataccacaggcacaatgcggctcactaacaatcaaaacagagccgagggaattagaaaaaagtacgggtagaagagggatattcagagatcagggcaagtctcccgagtctctgctctctcctctacctgatagaccaggacaaacatggccacctttacagatgcagagatcgacgagctatttgagacaagtggaactgtcattgacaacataattacagcccagggtaaaccagcagagactgttggaaggagtgcaatcccacaaggcaagaccaaggtgctgagcgcagcatgggagaagcatgggagcatccagccaccggccagtcaagacaaccccgatcgacaggacagatctgacaaacaaccatccacacccgagcaaacgaccccgcatgacagcccgccggccacatccgccgaccagccccccacccaggccacagacgaagccgtcgacacacagttcaggaccggagcaagcaactctctgctgttgatgcttgacaagctcagcaataaatcgtccaatgctaaaaagggcccatggtcgagcccccaagaggggaatcaccaacgtccgactcaacagcaggggagtcaacccagtcgcggaaacagtcaggaaagaccgcagaaccaagtcaaggccgcccctggaaaccagggcacagacgtgaacacagcatatcatggacaatgggaggagtcacaactatcagctggtgcaacccctcatgctctccgatcaaggcagagccaagacaatacccttgtatctgcggatcatgtccagccacctgtagactttgtgcaagcgatgatgtctatgatggaggcgatatcacagagagtaagtaaggttgactatcagctagatcttgtcttgaaacagacatcctccatccctatgatgcggtccgaaatccaacagctgaaaacatctgttgcagtcatggaagccaacttgggaatgatgaagattctggatcccggttgtgccaacatttcatctctgagtgatctacgggcagttgcccgatctcacccggttttagtttcaggccctggagacccctctccctatgtgacacaaggaggcgaaatggcacttaataaactttcgcaaccagtgccacatccatctgaattgattaaacccgccactgcatgcgggcctgatataggagtggaaaaggacactgtccgtgcattgatcatgtcacgcccaatgcacccgagttcttcagccaagctcctaagcaagttagatgcagccgggtcgatcgaggaaatcaggaaaatcaagcgccttgctctaaatggctaattactactgccacacgtagcgggtccctgtccactcggcatcacacggaatctgcaccgagttcccccccgcagacccaaggtccaactctccaagcggcaatcctctctcgcttcctcagccccactgaatggccggccaaccgtaattaatctagctacatttaagattaagaaaaaatacgggtagaattggagtgccccaattgtgccaagatggactcatctaggacaattgggctgtactttgattctgcccattcttctagcaacctgttagcatttccgatcgtcctacaaggcacaggagatgggaagaagcaaatcgccccgcaatataggatccagcgccttgacttgtggactgatagtaaggaggactcagtattcatcaccacctatggattcatctttcaagttgggaatgaagaagccactgtcggcatgatcgatgataaacccaagcgcgagttactttccgctgcgatgctctgcctaggaagcgtcccaaataccggagaccttattgagctggcaagggcctgtctcactatgatagtcacatgcaagaagagtgcaactaatactgagagaatggttttctcagtagtgcaggcaccccaagtgctgcaaagctgtagggttgtggcaaacaaatactcatcagtgaatgcagtcaagcacgtgaaagcgccagagaagattcccgggagtggaaccctagaatacaaggtgaactttgtctccttgactgtggtaccgaagaaggatgtctacaagatcccagctgcagtattgaaggtttctggctcgagtctgtacaatcttgcgctcaatgtcactattaatgtggaggtagacccgaggagtcctttggttaaatctttgtctaagtctgacagcggatactatgctaacctcttcttgcatattggacttatgaccaccgtagataggaaggggaagaaagtgacatttgacaagctggaaaagaaaataaggagccttgatctatctgtcgggctcagtgatgtgctcgggccttccgtgttggtaaaagcaagaggtgcacggactaagcttttggcacctttcttctctagcagtgggacagcctgctatcccatagcaaatgcttctcctcaggtggccaagatactctggagtcaaaccgcgtgcctgcggagcgttaaaatcattatccaagcaggtacccaacgcgctgtcgcagtgaccgccgaccacgaggttacctctactaagctggagaaggggcacacccttgccaaatacaatccttttaagaaataagctgcgtctctgagattgcgctccgcccactcacccagatcatcatgacacaaaaaactaatctgtcttgattatttacagttagtttacgcgtctatcaagttagaaaaaacacgggtagaagattctggatcccggttggcgccctccaggtgcaagatgggctccagaccttctaccaagaacccagcacctatgatgctgactatccgggttgcgctggtactgagttgcatctgtccggcaaactccattgatggcaggcctcttgcagctgcaggaattgtggttacaggagacaaagccgtcaacatatacacctcatcccagacaggatcaatcatagttaagctcctcccgaatctgcccaaggataaggaggcatgtgcgaaagcccccttggatgcatacaacaggacattgaccactttgctcaccccccttggtgactctatccgtaggatacaagagtctgtgactacatctggaggggggagacaggggcgccttataggcgccattattggcggtgtggctcttggggttgcaactgccgcacaaataacagcggccgcagctctgatacaagccaaacaaaatgctgccaacatcctccgacttaaagagagcattgccgcaaccaatgaggctgtgcatgaggtcactgacggattatcgcaactagcagtggcagttgggaagatgcagcagtttgttaatgaccaatttaataaaacagctcaggaattagactgcatcaaaattgcacagcaagttggtgtagagctcaacctgtacctaaccgaattgactacagtattcggaccacaaatcacttcacctgctttaaacaagctgactattcaggcactttacaatctagctggtggaaatatggattacttattgactaagttaggtgtagggaacaatcaactcagctcattaatcggtagcggcttaatcaccggtaaccctattctatacgactcacagactcaactcttgggtatacaggtaactctaccttcagtcgggaacctaaataatatgcgtgccacctacttggaaaccttatccgtaagcacaaccaggggatttgcctcggcacttgtccccaaagtggtgacacaggtcggttctgtgatagaagaacttgacacctcatactgtatagaaactgacttagatttatattgtacaagaatagtaacgttccctatgtcccctggtatttattcctgcttgagcggcaatacgtcggcctgtatgtactcaaagaccgaaggcgcacttactacaccatacatgactatcaaaggttcagtcatcgccaactgcaagatgacaacatgtagatgtgtaaaccccccgggtatcatatcgcaaaactatggagaagccgtgtctctaatagataaacaatcatgcaatgttttatccttaggcgggataactttaaggctcagtggggaattcgatgtaacttatcagaagaatatctcaatacaagattctcaagtaataataacaggcaatcttgatatctcaactgagcttgggaatgtcaacaactcgatcagtaatgctttgaataagttagaggaaagcaacagaaaactagacaaagtcaatgtcaaactgactagcacatctgctctcattacctatatcgttttgactatcatatctcttgtttttggtatacttagcctgattctagcatgctacctaatgtacaagcaaaaggcgcaacaaaagaccttattatggcttgggaataatactctagatcagatgagagccactacaaaaatgtgaacacagatgaggaacgaaggtttccctaatagttaattaagtgaaagttctggtagtctgtcagttcagagagttaagaaaaaactaccggttgtagatgaccaaaggacgatatacgggtagaacggtaagagaggccgcccctcaattgcgagccaggcttcacaacctccgttctaccgcttcaccgacaacagtcctcaatcatggaccgcgccgttagccaagttgcgttagagaatgatgaaagagaggcaaaaaatacatggcgcttgatattccggattgcaatcttattcttaacagtagtgaccttggctatatctgtagcctcccttttatatagcatgggggctagcacacctagcgatcttgtaggcataccgactaggatttccagggcagaagaaaagattacatctacacttggttccaatcaagatgtagtagataggatatataagcaagtggcccttgagtctccgttggcattgttaaatactgagaccacaattatgaacgcaataacatctctctcttatcagattaatggagctgcaaacaacagtgggtggggggcacctatccatgacccagattatataggggggataggcaaagaactcattgtagatgatgctagtgatgtcacatcattctatccctctgcatttcaagaacatctgaattttatcccggcgcctactacaggatcaggttgcactcgaataccctcatttgacatgagtgctacccattactgctacacccataatgtaatattgtctggatgcagagatcactcacattcatatcagtatttagcacttggtgtgctccggacatctgcaacagggagggtattcttttctactctgcgttccatcaacctggacgacacccaaaatcggaagtcttgcagtgtgagtgcaactcccctgggttgtgatatgctgtgctcgaaagtcacggagacagaggaagaagattataactcagctgtccctacgcggatggtacatgggaggttagggttcgacggccagtaccacgaaaaggacctagatgtcacaacattattcggggactgggtggccaactacccaggagtagggggtggatcttttattgacagccgcgtatggttctcagtctacggagggttaaaacccaattcacccagtgacactgtacaggaagggaaatatgtgatatacaagcgatacaatgacacatgcccagatgagcaagactaccagattcgaatggccaagtcttcgtataagcctggacggtttggtgggaaacgcatacagcaggctatcttatctatcaaggtgtcaacatccttaggcgaagacccggtactgactgtaccgcccaacacagtcacactcatgggggccgaaggcagaattctcacagtagggacatctcatttcttgtatcaacgagggtcatcatacttctctcccgcgttattatatcctatgacagtcagcaacaaaacagccactcttcatagtccttatacattcaatgccttcactcggccaggtagtatcccttgccaggcttcagcaagatgccccaactcgtgtgttactggagtctatacagatccatatcccctaatcttctatagaaaccacaccttgcgaggggtattcgggacaatgcttgatggtgtacaagcaagacttaaccctgcgtctgcagtattcgatagcacatcccgcagtcgcattactcgagtgagttcaagcagtaccaaagcagcatacacaacatcaacttgttttaaagtggtcaagactaataagacctattgtctcagcattgctgaaatatctaatactctcttcggagaattcagaatcgtcccgttactagttgagatcctcaaagatgacggggttagagaagccaggtctggctagttgagtcaattataaaggagttggaaagatggcattgtatcacctatcttctgcgacatcaagaatcaaaccgaatggccgcgcgggcccgaattccatgttgccagttgaccacaatcagccagtgctcatgcgatcagattaagccttgtcattaatctcttgattaagaaaaaatgtaagtggcaatgagatacaaggcaaaacagctcatggtaaataatacgggtaggacatggcgagctccggtcctgaaagggcagagcatcagattatcctaccagagccacacctgtcttcaccattggtcaagcacaaactactctattactggaaattaactgggctaccgcttcctgatgaatgtgacttcgaccacctcattctcagccgacaatggaaaaaaatacttgaatcggcctctcctgatactgagagaatgataaaactcggaagggcagtacaccaaactcttaaccacaattccagaataaccggagtgctccaccccaggtgtttagaacaactggctaatattgaggtcccagattcaaccaacaaatttcggaagattgagaagaagatccaaattcacaacacgagatatggagaactgttcacaaggctgtgtacgcatatagagaagaaactgctggggtcatcttggtctaacaatgtcccccggtcagaggagttcagcagcattcgtacggatccggcattctggtttcactcaaaatggtccacagccaagtttgcatggctccatataaaacagatccagaggcatctgatggtggcagctaagacaaggtctgcggccaacaaattggtgatgctaacccataaggtaggccaagtctttgtcactcctgaacttgtcgttgtgacgcatacgaatgagaacaagttcacatgtcttacccaggaacttgtattgatgtatgcagatatgatggagggcagagatatggtcaacataatatcaaccacggcggtgcatctcagaagcttatcagagaaaattgatgacattttgcggttaatagacgctctggcaaaagacttgggtaatcaagtctacgatgttgtatcactaatggagggatttgcatacggagctgtccagctactcgagccgtcaggtacatttgcaggagatttcttcgcattcaacctgcaggagcttaaagacattctaattggcctcctccccaatgatatagcagaatccgtgactcatgcaatcgctactgtattctctggtttagaacagaatcaagcagctgagatgttgtgtctgttgcgtctgtggggtcacccactgcttgagtcccgtattgcagcaaaggcagtcaggagccaaatgtgcgcaccgaaaatggtagactttgatatgatccttcaggtactgtctttcttcaagggaacaatcatcaacgggtacagaaagaagaatgcaggtgtgtggccgcgagtcaaagtggatacaatatatgggaaggtcattgggcaactacatgcagattcagcagagatttcacacgatatcatgttgagagagtataagagtttatctgcacttgaatttgagccatgtatagaatatgaccctgtcaccaacctgagcatgttcctaaaagacaaggcaatcgcacaccccaacgataattggcttgcctcgtttaggcggaaccttctctccgaagaccagaagaaacatgtaaaagaagcaacttcgactaatcgcctcttgatagagtttttagagtcaaatgattttgatccatataaagagatggaatatctgacgacccttgagtaccttagagatgacaatgtggcagtatcatactcgctcaaggagaaggaagtgaaagttaatggacggatcttcgctaagctgacaaagaagttaaggaactgtcaggtgatggcggaagggatcctagccgatcagattgcacctttctttcagggaaatggagtcattcaggatagcatatccttgaccaagagtatgctagcgatgagtcaactgtcttttaacagcaataagaaacgtatcactgactgtaaagaaagagtatcttcaaaccgcaatcatgatccgaaaagcaagaaccgtcggagagttgcaaccttcataacaactgacctgcaaaagtactgtcttaattggagatatcagacaatcaaattgttcgctcatgccatcaatcagttgatgggcctacctcacttcttcgaatggattcacctaagactgatggacactacgatgttcgtaggagaccctttcaatcctccaagtgaccctactgactgtgacctctcaagagtccctaatgatgacatatatattgtcagtgccagagggggtatcgaaggattatgccagaagctatggacaatgatctcaattgctgcaatccaacttgctgcagctagatcgcattgtcgtgttgcctgtatggtacagggtgataatcaagtaatagcagtaacgagagaggtaagatcagacgactctccggagatggtgttgacacagttgcatcaagccagtgataatttcttcaaggaattaattcatgtcaatcatttgattggccataatttgaaggatcgtgaaaccatcaggtcagacacattcttcatatacagcaaacgaatcttcaaagatggagcaatcctcagtcaagtcctcaaaaattcatctaaattagtgctagtgtcaggtgatctcagtgaaaacaccgtaatgtcctgtgccaacattgcctctactgtagcacggctatgcgagaacgggcttcccaaagacttctgttactatttaaactatataatgagttgtgtgcagacatactttgactctgagttctccatcaccaacaattcgcaccccgatcttaatcagtcgtggattgaggacatctcttttgtgcactcatatgttctgactcctgcccaattagggggactgagtaaccttcaatactcaaggctctacactagaaatatcggtgacccggggactactgcttttgcagagatcaagcgactagaagcagtgggattactgagtcctaacattatgactaatatcttaactaggccgcctgggaatggagattgggccagtctgtgcaacgacccatactctttcaattttgagactgttgcaagcccaaatattgttcttaagaaacatacgcaaagagtcctatttgaaacttgttcaaatcccttattgtctggagtgcacacagaggataatgaggcagaagagaaggcattggctgaattcttgcttaatcaagaggtgattcatccccgcgttgcgcatgccatcatggaggcaagctctgtaggtaggagaaagcaaattcaagggcttgttgacacaacaaacaccgtaattaagattgcgcttactaggaggccattaggcatcaagaggctgatgcggatagtcaattattctagcatgcatgcaatgctgtttagagacgatgttttttcctccagtagatccaaccaccccttagtctcttctaatatgtgttctctgacactggcagactatgcacggaatagaagctggtcacctttgacgggaggcaggaaaatactgggtgtatctaatcctgatacgatagaactcgtagagggtgagattcttagtgtaagcggagggtgtacaagatgtgacagcggagatgaacaatttacttggttccatcttccaagcaatatagaattgaccgatgacaccagcaagaatcctccgatgagggtaccatatctcgggtcaaagacacaggagaggagagctgcctcacttgcaaaaatagctcatatgtcgccacatgtaaaggctgccctaagggcatcatccgtgttgatctgggcttatggggataatgaagtaaattggactgctgctcttacgattgcaaaatctcggtgtaatgtaaacttagagtatcttcggttactgtcccctttacccacggctgggaatcttcaacatagactagatgatggtataactcagatgacattcacccctgcatctctctacagggtgtcaccttacattcacatatccaatgattctcaaaggctgttcactgaagaaggagtcaaagaggggaatgtggtttaccaacagatcatgctcttgggtttatctctaatcgaatcgatctttccaatgacaacaaccaggacatatgatgagatcacactgcacctacatagtaaatttagttgctgtatcagagaagcacctgttgcggttcctttcgagctacttggggtggtaccggaactgaggacagtgacctcaaataagtttatgtatgatcctagccctgtatcggagggagactttgcgagacttgacttagctatcttcaagagttatgagcttaatctggagtcatatcccacgatagagctaatgaacattctttcaatatccagcgggaagttgattggccagtctgtggtttcttatgatgaagatacctccataaagaatgacgccataatagtgtatgacaatacccgaaattggatcagtgaagctcagaattcagatgtggtccgcctatttgaatatgcagcacttgaagtgctcctcgactgttcttaccaactctattacctgagagtaagaggcctagacaatattgtcttatatatgggtgatttatacaagaatatgccaggaattctactttccaacattgcagctacaatatctcatcccgtcattcattcaaggttacatgcagtgggcctggtcaaccatgacggatcacaccaacttgcagatacggattttatcgaaatgtctgcaaaactattagtatcttgcacccgacgtgtgatctccggcttatattcaggaaataagtatgatctgctgttcccatctgtcttagatgataacctgaatgagaagatgcttcagctgatatcccggttatgctgtctgtacacggtactctttgctacaacaagagaaatcccgaaaataagaggcttaactgcagaagagaaatgttcaatactcactgagtatttactgtcggatgctgtgaaaccattacttagccccgatcaagtgagctctatcatgtctcctaacataattacattcccagctaatctgtactacatgtctcggaagagcctcaatttgatcagggaaagggaggacagggatactatcctggcgttgttgttcccccaagagccattattagagttcccttctgtgcaagatattggtgctcgagtgaaagatccattcacccgacaacctgcggcatttttgcaagagttagatttgagtgctccagcaaggtatgacgcattcacacttagtcagattcatcctgaactcacatctccaaatccggaggaagactacttagtacgatacttgttcagagggatagggactgcatcttcctcttggtataaggcatctcatctcctttctgtacccgaggtaagatgtgcaagacacgggaactccttatacttagctgaagggagcggagccatcatgagtcttctcgaactgcatgtaccacatgaaactatctattacaatacgctcttttcaaatgagatgaaccccccgcaacgacatttcgggccgaccccaactcagtttttgaattcggttgtttataggaatctacaggcggaggtaacatgcaaagatggatttgtccaagagttccgtccattatggagagaaaatacagaggaaagtgacctgacctcagataaagcagtggggtatattacatctgcagtgccctacagatctgtatcattgctgcattgtgacattgaaattcctccagggtccaatcaaagcttactagatcaactagctatcaatttatctctgattgccatgcattctgtaagggagggcggggtagtaatcatcaaagtgttgtatgcaatgggatactactttcatctactcatgaacttgtttgctccgtgttccacaaaaggatatattctctctaatggttatgcatgtcgaggagatatggagtgttacctggtatttgtcatgggttacctgggcgggcctacatttgtacatgaggtggtgaggatggcaaaaactctggtgcagcggcacggtacgctcttgtctaaatcagatgagatcacactgaccaggttattcacctcacagcggcagcgtgtgacagacatcctatccagtcctttaccaagattaataaagtacttgaggaagaatattgacactgcgctgattgaagccgggggacagcccgtccgtccattctgtgcggagagtctggtgagcacgctagcgaacataactcagataacccagattatcgctagtcacattgacacagttatccggtctgtgatatatatggaagctgagggtgatctcgctgacacagtatttctatttaccccttacaatctctctactgacgggaaaaagaggacatcacttatacagtgcacgagacagatcctagaggttacaatactaggtcttagagtcgaaaatctcaataaaataggcgatataatcagcctagtgcttaaaggcatgatctccatggaggaccttatcccactaaggacatacttgaagcatagtacctgccctaaatatttgaaggctgtcctaggtattaccaaactcaaagaaatgtttacagacacttctgtattgtacttgactcgtgctcaacaaaaattctacatgaaaactataggcaatgcagtcaaaggatattacagtaactgtgactcttaacgaaaatcacatattaataggctccttttttggccaattgtattcttgttgatttaatcatattatgttagaaaaaagttgaaccctgactccttaggactcgaattcgaactcaaataaatgtcttaaaaaaaggttgcgcacaattattcttgagtgtagtctcgtcattcaccaaatctttgtttggt

SEQ ID NO: 17 - protein, 539 aa, Human metapneumovirus
MSWKVVIIFSLLITPQHGLKESYLEESCSTITEGYLSVLRTGWYTNVFTLEVGDVENLTCADGPSLIKTELDLTKSALRELRTVSADQLAREEQIENPRQSRFVLGAIALGVATAAAVTAGVAIAKTIRLESEVTAIKNALKKTNEAVSTLGNGVRVLATAVRELKDFVSKNLTRAINKNKCDIADLKMAVSFSQFNRRFLNVVRQFSDNAGITPAISLDLMTDAELARAVSNMPTSAGQIKLMLENRAMVRRKGFGFLIGVYGSSVIYMVQLPIFGVIDTPCWIVKAAPSCSGKKGNYACLLREDQGWYCQNAGSTVYYPNEKDCETRGDHVFCDTAAGINVAEQSKECNINISTTNYPCKVSTGRHPISMVALSPLGALVACYKGVSCSIGSNRVGIIKQLNKGCSYITNQDADTVTIDNTVYQLSKVEGEQHVIKGRPVSSSFDPVKFPEDQFNVALDQVFESIENSQALVDQSNRILSSAEKGNTGFIIVIILIAVLGSTMILVSVFIIIKKTKKPTGAPPELSGVTNNGFIPHN

SEQ ID NO: 18 - protein, 539 aa, Human metapneumovirus
MSWKVVIIFSLLITPQHGLKESYLEESCSTITEGYLSVLRTGWYTNVFTLEVGDVENLTCSDGPSLIKTELDLTKSALRELKTVSADQLAREEQIENPRQSRFVLGAIALGVAAAAAVTAGVAIAKTIRLESEVTAINNALKKTNEAVSTLGNGVRVLATAVRELKDFVSKNLTRAINKNKCDIDDLKMAVSFSQFNRRFLNVVRQFSDNAGITPAISLDLMTDAELARAVPNMPTSAGQIKLMLENRAMVRRKGFGILIGVYGSSVIYMVQLPIFGVIDTPCWIVKAAPSCSEKKGNYACLLREDQGWYCQNAGSTVYYPNEKDCETRGDHVFCDTAAGINVAEQSKECNINISTTNYPCKVSTGRHPISMVALSPLGALVACYKGVSCSIGSNRVGIIKQLNKGCSYITNQDADTVTIDNTVYQLSKVEGEQHVIKGRPVSSSFDPIKFPEDQFNVALDQVFENIENSQALVDQSNRILSSAEKGNTGFIIVIILIAVLGSSMILVSIFIIIKKTKKPTGAPPELSGVTNNGFIPHN

SEQ ID NO: 19 - protein, 539 aa, Human metapneumovirus
MSWKVMIIISLLITPQHGLKESYLEESCSTITEGYLSVLRTGWYTNVFTLEVGDVENLTCTDGPSLIKTELDLTKSALRELKTVSADQLAREEQIENPRQSRFVLGAIALGVATAAAVTAGIAIAKTIRLESEVNAIKGALKQTNEAVSTLGNGVRVLATAVRELKEFVSKNLTSAINRNKCDIADLKMAVSFSQFNRRFLNVVRQFSDNAGITPAISLDLMTDAELARAVSYMPTSAGQIKLMLENRAMVRRKGFGILIGVYGSSVIYMVQLPIFGVIDTPCWIIKAAPSCSEKNGNYACLLREDQGWYCKNAGSTVYYPNEKDCETRGDHVFCDTAAGINVAEQSRECNINISTTNYPCKVSTGRHPISMVALSPLGALVACYKGVSCSIGSNWVGIIKQLPKGCSYITNQDADTVTIDNTVYQLSKVEGEQHVIKGRPVSSSFDPIKFPEDQFNVALDQVFESIENSQALVDQSNKILNSAEKGNTGFIIVVILVAVLGLTMISVSIIIIIKKTRKPTGAPPELNGVTNGGFIPHS

SEQ ID NO: 20 - protein, 539 aa, Human metapneumovirus
MSWKVMIIISLLITPQHGLKESYLEESCSTITEGYLSVLRTGWYTNVFTLEVGDVENLTCTDGPSLIKTELDLTKSALRELKTVSADQLAREEQIENPRQSRFVLGAIALGVATAAAVTAGIAIAKTIRLESEVNAIKGALKTTNEAVSTLGNGVRVLATAVRELKEFVSKNLTSAINKNKCDIADLKMAVSFSQFNRRFLNVVRQFSDNAGITPAISLDLMNDAELARAVSYMPTSAGQIKLMLENRAMVRRKGFGILIGVYGSSVIYMVQLPIFGVINTPCWIIKAAPSCSEKDGNYACLLREDQGWYCKNAGSTVYYPNEKDCETRGDHVFCDTAAGINVAEQSRECNINISTTNYPCKVSTGRHPISMVALSPLGALVACYKGVSCSTGSNQVGIIKQLPKGCSYITNQDADTVTIDNTVYQLSKVEGEQHVIKGRPVSNSFDPIRFPEDQFNVALDQVFESIENSQALVDQSNKILNSAEKGNTGFIIVIILIAVLGLTMISVSIIIIIKKTRKPAGAPPELNGVTNGGFIPHS

SEQ ID NO: 21 - protein, 574 aa, respiratory syncytial virus
MELLILKANAITTILTAVTFCFASGQNITEEFYQSTCSAVSKGYLSALRTGWYTSVITIELSNIKENKCNGTDAKVKLIKQELDKYKNAVTELQLLMQSTPPTNNRARRELPRFMNYTLNNAKKTNVTLSKKRKRRFLGFLLGVGSAIASGVAVSKVLHLEGEVNKIKSALLSTNKAVVSLSNGVSVLTSKVLDLKNYIDKQLLPIVNKQSCSISNIETVIEFQQKNNRLLEITREFSVNAGVTTPVSTYMLTNSELLSLINDMPITNDQKKLMSNNVQIVRQQSYSIMSIIKEEVLAYVVQLPLYGVIDTPCWKLHTSPLCTTNTKEGSNICLTRTDRGWYCDNAGSVSFFPQAETCKVQSNRVFCDTMNSLTLPSEINLCNVDIFNPKYDCKIMTSKTDVSSSVITSLGAIVSCYGKTKCTASNKNRGIIKTFSNGCDYVSNKGMDTVSVGNTLYYVNKQEGKSLYVKGEPIINFYDPLVFPSDEFDASISQVNEKINQSLAFIRKSDELLHNVNAGKSTTNIMITTIIIVIIVILLSLIAVGLLLYCKARSTPVTLSKDQLSGINNIAFSN

SEQ ID NO: 22 - protein, 254 aa, Human metapneumovirus
MESYLVDTYQGIPYTAAVQVDLIEKDLLPASLTIWFPLFQANTPPAVLLDQLKTLTITTLYAASQNGPILKVNASAQGAAMSVLPKKFEVNATVALDEYSKLEFDKLTVCEVKTVYLTTMKPYGMVSKFVSSAKSVGKKTHDLIALCDFMDLEKNTPVTIPAFIKSVSIKESESATVEAAISSEADQALTQAKIAPYAGLIMIMTMNNPKGIFKKLGAGTQVIVELGAYVQAESISKICKTWSHQGTRYVLKSR

SEQ ID NO: 23 - protein, 256 aa, respiratory syncytial virus
METYVNKLHEGSTYTAAVQYNVLEKDDDPASLTIWVPMFQSSMPADLLIKELANVNILVKQISTPKGPSLRVMINSRSAVLAQMPSKFTICANVSLDERSKLAYDVTTPCEIKACSLTCLKSKNMLTTVKDLTMKTLNPTHDIIALCEFENIVTSKKVIIPTYLRSISVRNKDLNTLENITTTEFKNAITNAKIIPYSGLLLVITVTDNKGAFKYIKPQSQFIVDLGAYLEKESIYYVTTNWKHTATRFAIKPMED

SEQ ID NO: 24 - DNA, 4361 bp, Artificial Sequence
  pBR322
ttctcatgtttgacagcttatcatcgataagctttaatgcggtagtttatcacagttaaattgctaacgcagtcaggcaccgtgtatgaaatctaacaatgcgctcatcgtcatcctcggcaccgtcaccctggatgctgtaggcataggcttggttatgccggtactgccgggcctcttgcgggatatcgtccattccgacagcatcgccagtcactatggcgtgctgctagcgctatatgcgttgatgcaatttctatgcgcacccgttctcggagcactgtccgaccgctttggccgccgcccagtcctgctcgcttcgctacttggagccactatcgactacgcgatcatggcgaccacacccgtcctgtggatcctctacgccggacgcatcgtggccggcatcaccggcgccacaggtgcggttgctggcgcctatatcgccgacatcaccgatggggaagatcgggctcgccacttcgggctcatgagcgcttgtttcggcgtgggtatggtggcaggccccgtggccgggggactgttgggcgccatctccttgcatgcaccattccttgcggcggcggtgctcaacggcctcaacctactactgggctgcttcctaatgcaggagtcgcataagggagagcgtcgaccgatgcccttgagagccttcaacccagtcagctccttccggtgggcgcggggcatgactatcgtcgccgcacttatgactgtcttctttatcatgcaactcgtaggacaggtgccggcagcgctctgggtcattttcggcgaggaccgctttcgctggagcgcgacgatgatcggcctgtcgcttgcggtattcggaatcttgcacgccctcgctcaagccttcgtcactggtcccgccaccaaacgtttcggcgagaagcaggccattatcgccggcatggcggccgacgcgctgggctacgtcttgctggcgttcgcgacgcgaggctggatggccttccccattatgattcttctcgcttccggcggcatcgggatgcccgcgttgcaggccatgctgtccaggcaggtagatgacgaccatcagggacagcttcaaggatcgctcgcggctcttaccagcctaacttcgatcactggaccgctgatcgtcacggcgatttatgccgcctcggcgagcacatggaacgggttggcatggattgtaggcgccgccctataccttgtctgcctccccgcgttgcgtcgcggtgcatggagccgggccacctcgacctgaatggaagccggcggcacctcgctaacggattcaccactccaagaattggagccaatcaattcttgcggagaactgtgaatgcgcaaaccaacccttggcagaacatatccatcgcgtccgccatctccagcagccgcacgcggcgcatctcgggcagcgttgggtcctggccacgggtgcgcatgatcgtgctcctgtcgttgaggacccggctaggctggcggggttgccttactggttagcagaatgaatcaccgatacgcgagcgaacgtgaagcgactgctgctgcaaaacgtctgcgacctgagcaacaacatgaatggtcttcggtttccgtgtttcgtaaagtctggaaacgcggaagtcagcgccctgcaccattatgttccggatctgcatcgcaggatgctgctggctaccctgtggaacacctacatctgtattaacgaagcgctggcattgaccctgagtgatttttctctggtcccgccgcatccataccgccagttgtttaccctcacaacgttccagtaaccgggcatgttcatcatcagtaacccgtatcgtgagcatcctctctcgtttcatcggtatcattacccccatgaacagaaatcccccttacacggaggcatcagtgaccaaacaggaaaaaaccgcccttaacatggcccgctttatcagaagccagacattaacgcttctggagaaactcaacgagctggacgcggatgaacaggcagacatctgtgaatcgcttcacgaccacgctgatgagctttaccgcagctgcctcgcgcgtttcggtgatgacggtgaaaacctctgacacatgcagctcccggagacggtcacagcttgtctgtaagcggatgccgggagcagacaagcccgtcagggcgcgtcagcgggtgttggcgggtgtcggggcgcagccatgacccagtcacgtagcgatagcggagtgtatactggcttaactatgcggcatcagagcagattgtactgagagtgcaccatatgcggtgtgaaataccgcacagatgcgtaaggagaaaataccgcatcaggcgctcttccgcttcctcgctcactgactcgctgcgctcggtcgttcggctgcggcgagcggtatcagctcactcaaaggcggtaatacggttatccacagaatcaggggataacgcaggaaagaacatgtgagcaaaaggccagcaaaaggccaggaaccgtaaaaaggccgcgttgctggcgtttttccataggctccgcccccctgacgagcatcacaaaaatcgacgctcaagtcagaggtggcgaaacccgacaggactataaagataccaggcgtttccccctggaagctccctcgtgcgctctcctgttccgaccctgccgcttaccggatacctgtccgcctttctcccttcgggaagcgtggcgctttctcatagctcacgctgtaggtatctcagttcggtgtaggtcgttcgctccaagctgggctgtgtgcacgaaccccccgttcagcccgaccgctgcgccttatccggtaactatcgtcttgagtccaacccggtaagacacgacttatcgccactggcagcagccactggtaacaggattagcagagcgaggtatgtaggcggtgctacagagttcttgaagtggtggcctaactacggctacactagaaggacagtatttggtatctgcgctctgctgaagccagttaccttcggaaaaagagttggtagctcttgatccggcaaacaaaccaccgctggtagcggtggtttttttgtttgcaagcagcagattacgcgcagaaaaaaaggatctcaagaagatcctttgatcttttctacggggtctgacgctcagtggaacgaaaactcacgttaagggattttggtcatgagattatcaaaaaggatcttcacctagatccttttaaattaaaaatgaagttttaaatcaatctaaagtatatatgagtaaacttggtctgacagttaccaatgcttaatcagtgaggcacctatctcagcgatctgtctatttcgttcatccatagttgcctgactccccgtcgtgtagataactacgatacgggagggcttaccatctggccccagtgctgcaatgataccgcgagacccacgctcaccggctccagatttatcagcaataaaccagccagccggaagggccgagcgcagaagtggtcctgcaactttatccgcctccatccagtctattaattgttgccgggaagctagagtaagtagttcgccagttaatagtttgcgcaacgttgttgccattgctgcaggcatcgtggtgtcacgctcgtcgtttggtatggcttcattcagctccggttcccaacgatcaaggcgagttacatgatcccccatgttgtgcaaaaaagcggttagctccttcggtcctccgatcgttgtcagaagtaagttggccgcagtgttatcactcatggttatggcagcactgcataattctcttactgtcatgccatccgtaagatgcttttctgtgactggtgagtactcaaccaagtcattctgagaatagtgtatgcggcgaccgagttgctcttgcccggcgtcaacacgggataataccgcgccacatagcagaactttaaaagtgctcatcattggaaaacgttcttcggggcgaaaactctcaaggatcttaccgctgttgagatccagttcgatgtaacccactcgtgcacccaactgatcttcagcatcttttactttcaccagcgtttctgggtgagcaaaaacaggaaggcaaaatgccgcaaaaaagggaataagggcgacacggaaatgttgaatactcatactcttcctttttcaatattattgaagcatttatcagggttattgtctcatgagcggatacatatttgaatgtatttagaaaaataaacaaataggggttccgcgcacatttccccgaaaagtgccacctgacgtctaagaaaccattattatcatgacattaacctataaaaataggcgtatcacgaggccctttcgtcttcaagaa

SEQ ID NO: 25 - DNA, 26 bp, Artificial Sequence
  ODN1a
  misc_feature (1)..(26): n=inosine
ncncncncncncncncncncncncnc

SEQ ID NO: 26 - protein, 11 aa, Artificial Sequence
  KLK peptide
KLKLLLLLKLK

SEQ ID NO: 27 - DNA, 1620 bp, Human metapneumovirus
atgtcttggaaagtggtgatcattttttcattgttaataacacctcaacacggtcttaaagagagctacttagaagagtcatgtagcactataactgaaggatatctcagtgttctgaggacaggttggtacaccaatgtttttacactggaggtaggcgatgtagagaaccttacatgtgccgatggacccagcttaataaaaacagaattagacctgaccaaaagtgcactaagagagctcagaacagtttctgctgatcaactggcaagagaggagcaaattgaaaatcccagacaatctagattcgttctaggagcaatagcactcggtgttgcaactgcagctgcagttacagcaggtgttgcaattgccaaaaccatccggcttgaaagtgaagtaacagcaattaagaatgccctcaaaaagaccaatgaagcagtatctacattggggaatggagttcgtgtgttggcaactgcagtgagagagctgaaagattttgtgagcaagaatctaacacgtgcaatcaacaaaaacaagtgcgacattgctgacctgaaaatggccgttagcttcagtcaattcaacagaaggttcctaaatgttgtgcggcaattttcagacaacgctggaataacaccagcaatatctttggacttaatgacagatgctgaactagccagagctgtttccaacatgccaacatctgcaggacaaataaaactgatgttggagaaccgtgcaatggtaagaagaaaagggttcggattcctgataggagtttacggaagctccgtaatttacatggtgcaactgccaatctttggggttatagacacgccttgctggatagtaaaagcagccccttcttgttcagaaaaaaagggaaactatgcttgcctcttaagagaagaccaaggatggtattgtcaaaatgcagggtcaactgtttactacccaaatgaaaaagactgtgaaacaagaggagaccatgtcttttgcgacacagcagcaggaatcaatgttgctgagcagtcaaaggagtgcaacataaacatatctactactaattacccatgcaaagttagcacaggaagacatcctatcagtatggttgcactatctcctcttggggctttggttgcttgctacaagggagtgagctgttccattggcagcaacagagtagggatcatcaagcaactgaacaaaggctgctcttatataaccaaccaagacgcagacacagtgacaatagacaacactgtataccagctaagcaaagttgaaggcgaacagcatgttataaaaggaaggccagtgtcaagcagctttgacccagtcaagtttcctgaagatcaattcaatgttgcacttgaccaagttttcgagagcattgagaacagtcaggccttggtggatcaatcaaacagaatcctaagcagtgcagagaaaggaaacactggcttcatcattgtaataattctaattgctgtccttggctctaccatgatcctagtgagtgtttttatcataataaagaaaacaaagaaacccacaggagcacctccagagctgagtggtgtcacaaacaatggcttcataccacataattag

SEQ ID NO: 28 - DNA, 1620 bp, Artificial Sequence
  optimized coding sequence
atgagctggaaggtggtcatcatcttcagcctgctgatcacccctcagcacggcctgaaagagagctacctggaagagtcctgcagcaccatcaccgagggctacctgagcgtgctgagaaccggctggtacaccaacgtgttcaccctggaagtgggcgacgtggaaaacctgacctgtgccgatggacccagcctgatcaagaccgagctggacctgacaaagagcgccctgagagagctgaggacagtctctgcagatcagctggccagagaggaacagatcgagaaccccagacagagcagattcgtgctgggagctatcgccctgggagttgctacagctgctgctgtgacagctggcgtggccattgccaagaccatccggctggaaagcgaagtgaccgccatcaagaacgccctgaaaaagaccaacgaggccgtgtctaccctcggcaatggcgttagagtgctggccacagccgtgcgcgagctgaaggatttcgtgtccaagaacctgaccagggccatcaacaagaacaagtgcgacattgccgacctgaagatggccgtgtccttcagccagttcaaccggcggttcctgaatgtcgtgcggcagttctctgacaacgccggcatcacaccagccatcagcctggatctgatgaccgatgccgaactggctagagccgtgtccaacatgcctacatctgccggccagatcaagctgatgctggaaaacagagccatggtccgacggaaaggcttcggctttctgatcggcgtgtacggcagcagcgtgatctacatggtgcagctgcctatcttcggcgtgatcgacaccccttgctggatcgtgaaagccgctcctagctgcagcgagaagaagggcaattacgcctgcctgctgagagaggaccaaggctggtactgtcagaatgccggcagcaccgtgtactaccccaacgagaaggactgcgagacaagaggcgaccacgtgttctgtgataccgccgctggaatcaacgtggccgagcagagcaaagagtgcaacatcaacatcagcaccacaaactacccctgcaaggtgtccaccggcagacaccctatcagcatggtggctctgtctccactgggagccctggtggcttgttataagggcgtgtcctgtagcatcggcagcaacagagtgggcatcatcaagcagctgaacaagggctgctcctacatcaccaaccaggacgccgataccgtgaccatcgacaataccgtgtatcagctgagcaaggtggaaggcgaacagcacgtgatcaagggcagacctgtgtccagcagcttcgaccccgtgaagttccccgaggaccagttcaatgtggccctggaccaggtgttcgagagcatcgagaatagccaggctctggtggaccagtccaaccggattctgtctagcgccgagaagggaaacaccggcttcatcatcgtgatcatcctgatcgccgtgctgggctccaccatgatcctggtgtccgtgttcatcatcatcaaaaagacgaagaagcccacaggcgcccctccagaactgtctggcgtgaccaacaatggcttcatccctcacaactag

SEQ ID NO: 29 - DNA, 1620 bp, Artificial Sequence
  optimized coding sequence
atgtcttggaaggtggtcatcatctttagcctgctgatcaccccacagcacggcctgaaggagagctacctggaggagtcctgttctaccatcacagagggctacctgtccgtgctgagaaccggctggtatacaaacgtgttcaccctggaggtcggcgatgtggagaatctgacatgcgccgacggcccttccctgatcaagacagagctggatctgaccaagagcgccctgagggagctgagaaccgtgtccgccgaccagctggccagggaggagcagatcgagaacccaaggcagtctcgctttgtgctgggagcaatcgccctgggagtggcaaccgccgccgccgtgaccgccggcgtggccatcgccaagacaatccgcctggagtctgaggtgaccgccatcaagaacgccctgaagaagacaaatgaggccgtgagcaccctgggaaacggcgtgcgggtgctggccacagccgtgagagagctgaaggatttcgtgtccaagaatctgacccgggccatcaacaagaataagtgtgacatcgccgatctgaagatggccgtgagcttctcccagtttaaccggagatttctgaatgtggtgagacagttctctgacaacgccggcatcacaccagccatcagcctggacctgatgaccgatgcagagctggccagggccgtgtctaacatgcccacaagcgccggccagatcaagctgatgctggagaatagggctatggtgcggaggaagggattcggctttctgatcggcgtgtacggcagctccgtgatctatatggtgcagctgcctatctttggcgtgatcgatacaccatgctggatcgtgaaggccgccccctcttgtagcgagaagaagggcaattacgcatgcctgctgagggaggatcagggatggtattgtcagaacgccggctccaccgtgtactatcccaatgagaaggactgtgagacaagaggcgaccacgtgttctgcgataccgccgccggcatcaacgtggcagagcagtccaaggagtgtaacatcaatatctctaccacaaattacccttgcaaggtgagcaccggcaggcaccctatcagcatggtggccctgtctccactgggcgccctggtggcctgctataagggcgtgtcctgttctatcggctccaaccgcgtgggcatcatcaagcagctgaacaagggctgctcttacatcacaaatcaggacgccgataccgtgacaatcgataataccgtgtatcagctgtccaaggtggagggagagcagcacgtgatcaagggacggcccgtgtctagctccttcgacccagtgaagtttcccgaggatcagttcaacgtggccctggaccaggtgtttgagagcatcgagaactcccaggccctggtggaccagagcaatagaatcctgagcagcgccgagaagggcaatacaggctttatcatcgtgatcatcctgatcgccgtgctgggcagcaccatgatcctggtgtccgtgttcatcatcatcaagaagacaaagaagccaaccggcgcccctcctgagctgagcggcgtgaccaacaatggcttcatccctcacaactag

SEQ ID NO: 30 - DNA, 1620 bp, Artificial Sequence
  optimized coding sequence
atgtcgtggaaggtcgtcatcatcttctcgctgctgatcacgccgcagcacggcctgaaagagtcgtacctcgaagagtcgtgctcgacgatcacggagggctacctgtcggtgctgcggacgggctggtacacgaacgtgttcacgctcgaagtcggcgacgtcgaaaacctgacgtgcgcggacggaccgtcgctgatcaagacggagctcgacctgacgaagtcggcgctgcgcgagctgcggacggtctcggcggatcagctcgcgcgcgaggaacagatcgagaacccgcggcagtcgcggttcgtgctcggcgcgatcgcgctcggcgtcgcgacggcggcggcggtgacggcgggcgtcgcgatcgcgaagacgatccggctcgaatcggaagtgacggcgatcaagaacgcgctgaaaaagacgaacgaggcggtgtcgacgctcggcaacggcgttcgcgtgctcgcgacggcggtgcgcgagctgaaggatttcgtgtcgaagaacctgacgcgcgcgatcaacaagaacaagtgcgacatcgcggacctgaagatggcggtgtcgttctcgcagttcaaccggcggttcctgaacgtcgtgcggcagttctcggacaacgcgggcatcacgccggcgatctcgctcgatctgatgacggacgcggaactcgcgcgcgcggtgtcgaacatgccgacgtcggcgggccagatcaagctgatgctcgaaaaccgcgcgatggtccgacggaaaggcttcggctttctgatcggcgtgtacggctcgtcggtgatctacatggtgcagctgccgatcttcggcgtgatcgacacgccgtgctggatcgtgaaagcggcgccgtcgtgctcggagaagaagggcaattacgcgtgcctgctgcgcgaggaccaaggctggtactgtcagaacgcgggctcgacggtgtactacccgaacgagaaggactgcgagacgcgcggcgaccacgtgttctgcgatacggcggcgggaatcaacgtcgcggagcagtcgaaagagtgcaacatcaacatctcgacgacgaactacccgtgcaaggtgtcgacgggccggcacccgatctcgatggtcgcgctgtcgccgctcggcgcgctcgtcgcgtgttataagggcgtgtcgtgttcgatcggctcgaaccgcgtcggcatcatcaagcagctgaacaagggctgctcgtacatcacgaaccaggacgcggatacggtgacgatcgacaatacggtgtatcagctgtcgaaggtcgaaggcgaacagcacgtgatcaagggccgcccggtgtcgtcgtcgttcgacccggtgaagttcccggaggaccagttcaacgtcgcgctcgaccaggtgttcgagtcgatcgagaattcgcaggcgctcgtcgaccagtcgaaccggattctgtcgtcggcggagaagggaaacacgggcttcatcatcgtgatcatcctgatcgcggtgctcggctcgacgatgatcctcgtgtcggtgttcatcatcatcaaaaagacgaagaagccgacgggcgcgccgccggaactgtcgggcgtgacgaacaacggcttcatcccgcacaactag

SEQ ID NO: 31 - DNA, 1659 bp, Artificial Sequence
  optimized coding sequence
atgggcagcagacccagcaccaagaatcccgctcctatgatgctgaccatcagagtggccctggtgctgagctgtatctgccccgccaatagcctgaaagagagctacctggaagagtcctgcagcaccatcaccgagggctacctgagcgtgctgagaaccggctggtacaccaacgtgttcaccctggaagtgggcgacgtggaaaacctgacctgtgccgatggacccagcctgatcaagaccgagctggacctgacaaagagcgccctgagagagctgaggacagtctctgcagatcagctggccagagaggaacagatcgagaaccccagacagagcagattcgtgctgggagctatcgccctgggagttgctacagctgctgctgtgacagctggcgtggccattgccaagaccatccggctggaaagcgaagtgaccgccatcaagaacgccctgaaaaagaccaacgaggccgtgtctaccctcggcaatggcgttagagtgctggccacagccgtgcgcgagctgaaggatttcgtgtccaagaacctgaccagggccatcaacaagaacaagtgcgacattgccgacctgaagatggccgtgtccttcagccagttcaaccggcggttcctgaatgtcgtgcggcagttctctgacaacgccggcatcacaccagccatcagcctggatctgatgaccgatgccgaactggctagagccgtgtccaacatgcctacatctgccggccagatcaagctgatgctggaaaacagagccatggtccgacggaaaggcttcggctttctgatcggcgtgtacggcagcagcgtgatctacatggtgcagctgcctatcttcggcgtgatcgacaccccttgctggatcgtgaaagccgctcctagctgcagcgagaagaagggcaattacgcctgcctgctgagagaggaccaaggctggtactgtcagaatgccggcagcaccgtgtactaccccaacgagaaggactgcgagacaagaggcgaccacgtgttctgtgataccgccgctggaatcaacgtggccgagcagagcaaagagtgcaacatcaacatcagcaccacaaactacccctgcaaggtgtccaccggcagacaccctatcagcatggtggctctgtctccactgggagccctggtggcttgttataagggcgtgtcctgtagcatcggcagcaacagagtgggcatcatcaagcagctgaacaagggctgctcctacatcaccaaccaggacgccgataccgtgaccatcgacaataccgtgtatcagctgagcaaggtggaaggcgaacagcacgtgatcaagggcagacctgtgtccagcagcttcgaccccgtgaagttccccgaggaccagttcaatgtggccctggaccaggtgttcgagagcatcgagaatagccaggctctggtggaccagtccaaccggattctgtctagcgccgagaagggaaacaccggcttcatcatcgtgatcatcctgatcgccgtgctgggctccaccatgatcctggtgtccgtgttcatcatcatcaaaaagacgaagaagcccacaggcgcccctccagaactgtctggcgtgaccaacaatggcttcatccctcacaactag

SEQ ID NO: 32 - DNA, 1620 bp, Artificial Sequence
  optimized coding sequence
atgagctggaaggtggtcatcatcttcagcctgctgatcacccctcagcatggcctgaaagagagctacctggaagagtcctgcagcaccatcacagagggctacctgagtgtgctgagaacaggctggtacaccaatgtgttcaccctggaagtgggggatgtggaaaacctgacctgtgctgatggacccagcctgatcaagacagagctggacctgacaaagagtgccctgagagagctgaggacagtctctgcagatcagctggccagagaggaacagattgagaaccccagacagagcagatttgtgctgggagctattgccctgggagttgctacagctgctgctgtgacagctggggtggccattgccaagaccatcagactggaaagtgaagtgacagccatcaagaatgccctgaaaaagaccaatgaggctgtgtctaccctgggcaatggggttagagtgctggccacagctgtgagagagctgaaggattttgtgtccaagaacctgaccagggccatcaacaagaacaagtgtgacattgctgacctgaagatggctgtgtccttcagccagttcaacagaagattcctgaatgtggtgagacagttctctgacaatgctggcatcacaccagccatcagcctggatctgatgacagatgctgaactggctagagctgtgtccaacatgcctacatctgctggccagatcaagctgatgctggaaaacagagccatggtcagaagaaaaggctttggctttctgattggggtgtatggcagcagtgtgatctacatggtgcagctgcctatctttggggtgattgacaccccttgctggattgtgaaagctgctcctagctgcagtgagaagaagggcaattatgcctgcctgctgagagaggaccaaggctggtactgtcagaatgctggcagcacagtgtactaccccaatgagaaggactgtgagacaagaggggaccatgtgttctgtgatacagctgctggaatcaatgtggctgagcagagcaaagagtgcaacatcaacatcagcaccacaaactacccctgcaaggtgtccacaggcagacaccctatcagcatggtggctctgtctccactgggagccctggtggcttgttataagggggtgtcctgtagcattggcagcaacagagtgggcatcatcaagcagctgaacaagggctgctcctacatcaccaaccaggatgctgatacagtgaccattgacaatacagtgtatcagctgagcaaggtggaaggggaacagcatgtgatcaagggcagacctgtgtccagcagctttgaccctgtgaagttccctgaggaccagttcaatgtggccctggaccaggtgtttgagagcattgagaatagccaggctctggtggaccagtccaacagaattctgtctagtgctgagaagggaaacacaggcttcatcattgtgatcatcctgattgctgtgctgggctccaccatgatcctggtgagtgtgttcatcatcatcaaaaagacaaagaagcccacaggggcccctccagaactgtctggggtgaccaacaatggcttcatccctcacaactag

SEQ ID NO: 33 - DNA, 734 bp, Artificial Sequence
  Artificial sequence
catggcgcgcctaagaaaaaatacgggtagaagccaccatgcccgccatgaagatcgagtgccgcatcaccggcaccctgaacggcgtggagttcgagctggtgggcggcggagagggcacccccgagcagggccgcatgaccaacaagatgaagagcaccaaaggcgccctgaccttcagcccctacctgctgagccacgtgatgggctacggcttctaccacttcggcacctaccccagcggctacgagaaccccttcctgcacgccatcaacaacggcggctacaccaacacccgcatcgagaagtacgaggacggcggcgtgctgcacgtgagcttcagctaccgctacgaggccggccgcgtgatcggcgacttcaaggtggtgggcaccggcttccccgaggacagcgtgatcttcaccgacaagatcatccgcagcaacgccaccgtggagcacctgcaccccatgggcgataacgtgctggtgggcagcttcgcccgcaccttcagcctgcgcgacggcggctactacagcttcgtggtggacagccacatgcacttcaagagcgccatccaccccagcatcctgcagaacgggggccccatgttcgccttccgccgcgtggaggagctgcacagcaacaccgagctgggcatcgtggagtaccagcacgccttcaagacccccatcgccttcgccagatctcgagctcgataggggcgcgccggc

SEQ ID NO: 34 - DNA, 894 bp, Human metapneumovirus
ggccgcgcgggccttaattaaacgcgtggccggccggcgcgcctaagaaaaaatacgggtagaagccaccatggagtcctacctagtagacacctatcaaggcattccttacacagcagctgttcaagttgatctaatagaaaaggacctgttacctgcaagcctaacaatatggttccctttgtttcaggccaacacaccaccagcagtgctgctcgatcagctaaaaaccctgacaataaccactctgtatgctgcatcacaaaatggtccaatactcaaagtgaatgcatcagcccaaggtgcagcaatgtctgtacttcccaaaaaatttgaagtcaatgcgactgtagcactcgatgaatatagcaaactggaatttgacaaactcacagtctgtgaagtaaaaacagtttacttaacaaccatgaaaccatacgggatggtatcaaaatttgtgagctcagccaaatcagttggcaaaaaaacacatgatctaatcgcactatgtgattttatggatctagaaaagaacacacctgttacaataccagcattcatcaaatcagtttcaatcaaagagagtgagtcagctactgttgaagctgctataagcagtgaagcagaccaagctctaacacaggccaaaattgcaccttatgcgggattaattatgatcatgactatgaacaatcccaaaggcatattcaaaaagcttggagctgggactcaagtcatagtagaactaggagcatatgtccaggctgaaagcataagcaaaatatgcaagacttggagccatcaagggacaagatatgtcttgaagtccagataatagataatggcgcgccatggccggccacgcgtaattaattaatataggccgcgcgggcc

SEQ ID NO: 35 - DNA, 750 bp, Cytomegalovirus
tcaatattggccattagccatattattcattggttatatagcataaatcaatattggctattggccattgcatacgttgtatctatatcataatatgtacatttatattggctcatgtccaatatgaccgccatgttggcattgattattgactagttattaatagtaatcaattacggggtcattagttcatagcccatatatggagttccgcgttacataacttacggtaaatggcccgcctggctgaccgcccaacgacccccgcccattgacgtcaataatgacgtatgttcccatagtaacgccaatagggactttccattgacgtcaatgggtggagtatttacggtaaactgcccacttggcagtacatcaagtgtatcatatgccaagtccgccccctattgacgtcaatgacggtaaatggcccgcctggcattatgcccagtacatgaccttacgggactttcctacttggcagtacatctacgtattagtcatcgctattaccatggtgatgcggttttggcagtacaccaatgggcgtggatagcggtttgactcacggggatttccaagtctccaccccattgacgtcaatgggagtttgttttggcaccaaaatcaacgggactttccaaaatgtcgtaacaactgcgatcgcccgccccgttgacgcaaatgggcggtaggcgtgtacggtgggaggtctatataagcagagctcgtttagtgaaccgtcagatc

SEQ ID NO: 36 - DNA, 534 bp, Artificial Sequence
  Artificial sequence
ggtaccatatctcgggtcaaagacacaggagaggagagctgcctcacttgcaaaaatagctcatatgtcgccacatgtaaaggctgccctaagggcatcatccgtgttgatctgggcttatggggataatgaagtaaattggactgctgctcttacgattgcaaaatctcggtgtaatgtaaacttagagtatcttcggttactgtcccctttacccacggctgggaatcttcaacatagactagatgatggtataactcagatgacattcacccctgcatctctctacagggtgtcaccttacattcacatatccaatgattctcaaaggctgttcactgaagaaggagtcaaagaggggaatgtggtttaccaacagatcatgctcttgggtttatctctaatcgaatcgatctttccaatgacaacaaccaggacatatgatgagatcacactgcacctacatagtaaatttagttgctgtatcagagaagcacctgttgcggttcctttcgagctacttggggtggtacc

SEQ ID NO: 37 - DNA, 1747 bp, Artificial Sequence
  Artificial sequence
ggccgcgcgggccattaattaataatacgcgtggccggccatggcgcgcctaagaaaaaatacgggtagaagccaccatgtcttggaaagtggtgatcattttttcattgttaataacacctcaacacggtcttaaagagagctacttagaagagtcatgtagcactataactgaaggatatctcagtgttctgaggacaggttggtacaccaatgtttttacactggaggtaggcgatgtagagaaccttacatgtgccgatggacccagcttaataaaaacagaattagacctgaccaaaagtgcactaagagagctcagaacagtttctgctgatcaactggcaagagaggagcaaattgaaaatcccagacaatctagattcgttctaggagcaatagcactcggtgttgcaactgcagctgcagttacagcaggtgttgcaattgccaaaaccatccggcttgaaagtgaagtaacagcaattaagaatgccctcaaaaagaccaatgaagcagtatctacattggggaatggagttcgtgtgttggcaactgcagtgagagagctgaaagattttgtgagcaagaatctaacacgtgcaatcaacaaaaacaagtgcgacattgctgacctgaaaatggccgttagcttcagtcaattcaacagaaggttcctaaatgttgtgcggcaattttcagacaacgctggaataacaccagcaatatctttggacttaatgacagatgctgaactagccagagctgtttccaacatgccaacatctgcaggacaaataaaactgatgttggagaaccgtgcaatggtaagaagaaaagggttcggattcctgataggagtttacggaagctccgtaatttacatggtgcaactgccaatctttggggttatagacacgccttgctggatagtaaaagcagccccttcttgttcagaaaaaaagggaaactatgcttgcctcttaagagaagaccaaggatggtattgtcaaaatgcagggtcaactgtttactacccaaatgaaaaagactgtgaaacaagaggagaccatgtcttttgcgacacagcagcaggaatcaatgttgctgagcagtcaaaggagtgcaacataaacatatctactactaattacccatgcaaagttagcacaggaagacatcctatcagtatggttgcactatctcctcttggggctttggttgcttgctacaagggagtgagctgttccattggcagcaacagagtagggatcatcaagcaactgaacaaaggctgctcttatataaccaaccaagacgcagacacagtgacaatagacaacactgtataccagctaagcaaagttgaaggcgaacagcatgttataaaaggaaggccagtgtcaagcagctttgacccagtcaagtttcctgaagatcaattcaatgttgcacttgaccaagttttcgagagcattgagaacagtcaggccttggtggatcaatcaaacagaatcctaagcagtgcagagaaaggaaacactggcttcatcattgtaataattctaattgctgtccttggctctaccatgatcctagtgagtgtttttatcataataaagaaaacaaagaaacccacaggagcacctccagagctgagtggtgtcacaaacaatggcttcataccacataattagaggcgcgccggccggccattaacgcgtttaattaataggccgcgcgggcc

SEQ ID NO: 38 - DNA, 5472 bp, Artificial Sequence
  Artificial sequence
tcaatattggccattagccatattattcattggttatatagcataaatcaatattggctattggccattgcatacgttgtatctatatcataatatgtacatttatattggctcatgtccaatatgaccgccatgttggcattgattattgactagttattaatagtaatcaattacggggtcattagttcatagcccatatatggagttccgcgttacataacttacggtaaatggcccgcctggctgaccgcccaacgacccccgcccattgacgtcaataatgacgtatgttcccatagtaacgccaatagggactttccattgacgtcaatgggtggagtatttacggtaaactgcccacttggcagtacatcaagtgtatcatatgccaagtccgccccctattgacgtcaatgacggtaaatggcccgcctggcattatgcccagtacatgaccttacgggactttcctacttggcagtacatctacgtattagtcatcgctattaccatggtgatgcggttttggcagtacaccaatgggcgtggatagcggtttgactcacggggatttccaagtctccaccccattgacgtcaatgggagtttgttttggcaccaaaatcaacgggactttccaaaatgtcgtaacaactgcgatcgcccgccccgttgacgcaaatgggcggtaggcgtgtacggtgggaggtctatataagcagagctcgtttagtgaaccgtcagatcactagaagctttattgcggtagtttatcacagttaaattgctaacgcagtcagtgcttctgacacaacagtctcgaacttaagctgcagtgactctcttaaggtagccttgcagaagttggtcgtgaggcactgggcaggtaagtatcaaggttacaagacaggtttaaggagaccaatagaaactgggcttgtcgagacagagaagactcttgcgtttctgataggcacctattggtcttactgacatccactttgcctttctctccacaggtgtccactcccagttcaattacagctcttaaggctagagtacttaatacgactcactataggctagcctcgagaattcacgcgtggtacctctagagtcgacccgggcggccgcttccctttagtgagggttaatgcttcgagcagacatgataagatacattgatgagtttggacaaaccacaactagaatgcagtgaaaaaaatgctttatttgtgaaatttgtgatgctattgctttatttgtaaccattataagctgcaataaacaagttaacaacaacaattgcattcattttatgtttcaggttcagggggagatgtgggaggttttttaaagcaagtaaaacctctacaaatgtggtaaaatccgataaggatcgatccgggctggcgtaatagcgaagaggcccgcaccgatcgcccttcccaacagttgcgcagcctgaatggcgaatggacgcgccctgtagcggcgcattaagcgcggcgggtgtggtggttacgcgcagcgtgaccgctacacttgccagcgccctagcgcccgctcctttcgctttcttcccttcctttctcgccacgttcgccggctttccccgtcaagctctaaatcgggggctccctttagggttccgatttagtgctttacggcacctcgaccccaaaaaacttgattagggtgatggttcacgtagtgggccatcgccctgatagacggtttttcgccctttgacgttggagtccacgttctttaatagtggactcttgttccaaactggaacaacactcaaccctatctcggtctattcttttgatttataagggattttgccgatttcggcctattggttaaaaaatgagctgatttaacaaaaatttaacgcgaattttaacaaaatattaacgcttacaatttcctgatgcggtattttctccttacgcatctgtgcggtatttcacaccgcatacgcggatctgcgcagcaccatggcctgaaataacctctgaaagaggaacttggttaggtaccttctgaggcggaaagaaccagctgtggaatgtgtgtcagttagggtgtggaaagtccccaggctccccagcaggcagaagtatgcaaagcatgcatctcaattagtcagcaaccaggtgtggaaagtccccaggctccccagcaggcagaagtatgcaaagcatgcatctcaattagtcagcaaccatagtcccgcccctaactccgcccatcccgcccctaactccgcccagttccgcccattctccgccccatggctgactaattttttttatttatgcagaggccgaggccgcctcggcctctgagctattccagaagtagtgaggaggcttttttggaggcctaggcttttgcaaaaagcttgattcttctgacacaacagtctcgaacttaaggctagagccaccatgattgaacaagatggattgcacgcaggttctccggccgcttgggtggagaggctattcggctatgactgggcacaacagacaatcggctgctctgatgccgccgtgttccggctgtcagcgcaggggcgcccggttctttttgtcaagaccgacctgtccggtgccctgaatgaactgcaggacgaggcagcgcggctatcgtggctggccacgacgggcgttccttgcgcagctgtgctcgacgttgtcactgaagcgggaagggactggctgctattgggcgaagtgccggggcaggatctcctgtcatctcaccttgctcctgccgagaaagtatccatcatggctgatgcaatgcggcggctgcatacgcttgatccggctacctgcccattcgaccaccaagcgaaacatcgcatcgagcgagcacgtactcggatggaagccggtcttgtcgatcaggatgatctggacgaagagcatcaggggctcgcgccagccgaactgttcgccaggctcaaggcgcgcatgcccgacggcgaggatctcgtcgtgacccatggcgatgcctgcttgccgaatatcatggtggaaaatggccgcttttctggattcatcgactgtggccggctgggtgtggcggaccgctatcaggacatagcgttggctacccgtgatattgctgaagagcttggcggcgaatgggctgaccgcttcctcgtgctttacggtatcgccgctcccgattcgcagcgcatcgccttctatcgccttcttgacgagttcttctgagcgggactctggggttcgaaatgaccgaccaagcgacgcccaacctgccatcacgatggccgcaataaaatatctttattttcattacatctgtgtgttggttttttgtgtgaatcgatagcgataaggatccgcgtatggtgcactctcagtacaatctgctctgatgccgcatagttaagccagccccgacacccgccaacacccgctgacgcgccctgacgggcttgtctgctcccggcatccgcttacagacaagctgtgaccgtctccgggagctgcatgtgtcagaggttttcaccgtcatcaccgaaacgcgcgagacgaaagggcctcgtgatacgcctatttttataggttaatgtcatgataataatggtttcttagacgtcaggtggcacttttcggggaaatgtgcgcggaacccctatttgtttatttttctaaatacattcaaatatgtatccgctcatgagacaataaccctgataaatgcttcaataatattgaaaaaggaagagtatgagtattcaacatttccgtgtcgcccttattcccttttttgcggcattttgccttcctgtttttgctcacccagaaacgctggtgaaagtaaaagatgctgaagatcagttgggtgcacgagtgggttacatcgaactggatctcaacagcggtaagatccttgagagttttcgccccgaagaacgttttccaatgatgagcacttttaaagttctgctatgtggcgcggtattatcccgtattgacgccgggcaagagcaactcggtcgccgcatacactattctcagaatgacttggttgagtactcaccagtcacagaaaagcatcttacggatggcatgacagtaagagaattatgcagtgctgccataaccatgagtgataacactgcggccaacttacttctgacaacgatcggaggaccgaaggagctaaccgcttttttgcacaacatgggggatcatgtaactcgccttgatcgttgggaaccggagctgaatgaagccataccaaacgacgagcgtgacaccacgatgcctgtagcaatggcaacaacgttgcgcaaactattaactggcgaactacttactctagcttcccggcaacaattaatagactggatggaggcggataaagttgcaggaccacttctgcgctcggcccttccggctggctggtttattgctgataaatctggagccggtgagcgtgggtctcgcggtatcattgcagcactggggccagatggtaagccctcccgtatcgtagttatctacacgacggggagtcaggcaactatggatgaacgaaatagacagatcgctgagataggtgcctcactgattaagcattggtaactgtcagaccaagtttactcatatatactttagattgatttaaaacttcatttttaatttaaaaggatctaggtgaagatcctttttgataatctcatgaccaaaatcccttaacgtgagttttcgttccactgagcgtcagaccccgtagaaaagatcaaaggatcttcttgagatcctttttttctgcgcgtaatctgctgcttgcaaacaaaaaaaccaccgctaccagcggtggtttgtttgccggatcaagagctaccaactctttttccgaaggtaactggcttcagcagagcgcagataccaaatactgttcttctagtgtagccgtagttaggccaccacttcaagaactctgtagcaccgcctacatacctcgctctgctaatcctgttaccagtggctgctgccagtggcgataagtcgtgtcttaccgggttggactcaagacgatagttaccggataaggcgcagcggtcgggctgaacggggggttcgtgcacacagcccagcttggagcgaacgacctacaccgaactgagatacctacagcgtgagctatgagaaagcgccacgcttcccgaagggagaaaggcggacaggtatccggtaagcggcagggtcggaacaggagagcgcacgagggagcttccagggggaaacgcctggtatctttatagtcctgtcgggtttcgccacctctgacttgagcgtcgatttttgtgatgctcgtcaggggggcggagcctatggaaaaacgccagcaacgcggcctttttacggttcctggccttttgctggccttttgctcacatggctcgacagatct

SEQ ID NO: 39 - DNA, 2892 bp, Artificial Sequence
  Artificial sequence
tcaatattggccattagccatattattcattggttatatagcataaatcaatattggctattggccattgcatacgttgtatctatatcataatatgtacatttatattggctcatgtccaatatgaccgccatgttggcattgattattgactagttattaatagtaatcaattacggggtcattagttcatagcccatatatggagttccgcgttacataacttacggtaaatggcccgcctggctgaccgcccaacgacccccgcccattgacgtcaataatgacgtatgttcccatagtaacgccaatagggactttccattgacgtcaatgggtggagtatttacggtaaactgcccacttggcagtacatcaagtgtatcatatgccaagtccgccccctattgacgtcaatgacggtaaatggcccgcctggcattatgcccagtacatgaccttacgggactttcctacttggcagtacatctacgtattagtcatcgctattaccatggtgatgcggttttggcagtacaccaatgggcgtggatagcggtttgactcacggggatttccaagtctccaccccattgacgtcaatgggagtttgttttggcaccaaaatcaacgggactttccaaaatgtcgtaacaactgcgatcgcccgccccgttgacgcaaatgggcggtaggcgtgtacggtgggaggtctatataagcagagctcgtttagtgaaccgtcagatcactagaagctttattgcggtagtttatcacagttaaattgctaacgcagtcagtgcttctgacacaacagtctcgaacttaagctgcagtgactctcttaaggtagccttgcagaagttggtcgtgaggcactgggcaggtaagtatcaaggttacaagacaggtttaaggagaccaatagaaactgggcttgtcgagacagagaagactcttgcgtttctgataggcacctattggtcttactgacatccactttgcctttctctccacaggtgtccactcccagttcaattacagctcttaaggctagagtacttaatacgactcactataggctagcctcgagaattccgagtgcgagcccgaagcacaaactcgagaaagccttctgccaacatgtcttccgtatttgatgagtacgaacagctcctcgcggctcagactcgccccaatggagctcatggagggggagaaaaagggagtaccttaaaagtagacgtcccggtattcactcttaacagtgatgacccagaagatagatggagctttgtggtattctgcctccggattgctgttagcgaagatgccaacaaaccactcaggcaaggtgctctcatatctcttttatgctcccactcacaggtaatgaggaaccatgttgccattgcagggaaacagaatgaagccacattggccgtgcttgagattgatggctttgccaacggcacgccccagttcaacaataggagtggagtgtctgaagagagagcacagagatttgcgatgatagcaggatctctccctcgggcatgcagcaacggaaccccgttcgtcacagccggggcagaagatgatgcaccagaagacatcaccgataccctggagaggatcctctctatccaggctcaagtatgggtcacagtagcaaaagccatgactgcgtatgagactgcagatgagtcggaaacaaggcgaatcaataagtatatgcagcaaggcagggtccaaaagaaatacatcctctaccccgtatgcaggagcacaatccaactcacgatcagacagtctcttgcagtccgcatctttttggttagcgagctcaagagaggccgcaacacggcaggtggtacctctacttattataacctggtaggggacgtagactcatacatcaggaataccgggcttactgcattcttcttgacactcaagtacggaatcaacaccaagacatcagcccttgcacttagtagcctctcaggcgacatccagaagatgaagcagctcatgcgtttgtatcggatgaaaggagataatgcgccgtacatgacattacttggtgatagtgaccagatgagctttgcgcctgccgagtatgcacaactttactcctttgccatgggtatggcatcagtcctagataaaggtactgggaaataccaatttgccagggactttatgagcacatcattctggagacttggagtagagtacgctcaggctcagggaagtagcattaacgaggatatggctgccgagctaaagctaaccccagcagcaatgaagggcctggcagctgctgcccaacgggtctccgacgataccagcagcatatacatgcctactcaacaagtcggagtcctcactgggcttagcgagggggggtcccaagctctacaaggcggatcgaatagatcgcaagggcaaccagaagccggggatggggagacccaattcctggatctgatgagagcggtagcaaatagcatgagggaggcgccaaactctgcacagggcactccccaatcggggcctcccccaactcctgggccatcccaagataacgacaccgactgggggtattgacctgcaggcatgcaagggcggccgcttccctttagtgagggttaatgcttcgagcagacatgataagatacattgatgagtttggacaaaccacaactagaatgcagtgaaaaaaatgctttatttgtgaaatttgtgatgctattgctttatttgtaaccattataagctgcaataaacaagttaacaacaacaattgcattcattttatgtttcaggttcagggggagatgtgggaggttttttaaagcaagtaaaacctctacaaatgtggta

SEQ ID NO: 40 - DNA, 2658 bp, Artificial Sequence
  Artificial sequence
tcaatattggccattagccatattattcattggttatatagcataaatcaatattggctattggccattgcatacgttgtatctatatcataatatgtacatttatattggctcatgtccaatatgaccgccatgttggcattgattattgactagttattaatagtaatcaattacggggtcattagttcatagcccatatatggagttccgcgttacataacttacggtaaatggcccgcctggctgaccgcccaacgacccccgcccattgacgtcaataatgacgtatgttcccatagtaacgccaatagggactttccattgacgtcaatgggtggagtatttacggtaaactgcccacttggcagtacatcaagtgtatcatatgccaagtccgccccctattgacgtcaatgacggtaaatggcccgcctggcattatgcccagtacatgaccttacgggactttcctacttggcagtacatctacgtattagtcatcgctattaccatggtgatgcggttttggcagtacaccaatgggcgtggatagcggtttgactcacggggatttccaagtctccaccccattgacgtcaatgggagtttgttttggcaccaaaatcaacgggactttccaaaatgtcgtaacaactgcgatcgcccgccccgttgacgcaaatgggcggtaggcgtgtacggtgggaggtctatataagcagagctcgtttagtgaaccgtcagatcactagaagctttattgcggtagtttatcacagttaaattgctaacgcagtcagtgcttctgacacaacagtctcgaacttaagctgcagtgactctcttaaggtagccttgcagaagttggtcgtgaggcactgggcaggtaagtatcaaggttacaagacaggtttaaggagaccaatagaaactgggcttgtcgagacagagaagactcttgcgtttctgataggcacctattggtcttactgacatccactttgcctttctctccacaggtgtccactcccagttcaattacagctcttaaggctagagtacttaatacgactcactataggctagcctcgagaattcagaaaaaagtacgggtagaagagggatattcagagatcagggcaagtctcccgagtctctgctctctcctctacctgatagaccaggacaaacaatggccacctttacagatgcagagatcgacgagctatttgagacaagtggaactgtcattgacaacataattacagcccagggtaaaccagcagagactgttggaaggagtgcaatcccacaaggcaagaccaaggtgctgagcgcagcatgggagaagcatgggagcatccagccaccggccagtcaagacaaccccgatcgacaggacagatctgacaaacaaccatccacacccgagcaaacgaccccgcatgacagcccgccggccacatccgccgaccagccccccacccaggccacagacgaagccgtcgacacacagctcaggaccggagcaagcaactctctgctgttgatgcttgacaagctcagcaataaatcgtccaatgctaaaaagggcccatggtcgagcccccaagaggggaatcaccaacgtccgactcaacagcaggggagtcaacccagtcgcggaaacagtcaggaaagaccgcagaaccaagtcaaggccgcccctggaaaccagggcacagacgtgaacacagcatatcatggacaatgggaggagtcacaactatcagctggtgcaacccctcatgctctccgatcaaggcagagccaagacaatacccttgtatctgcggatcatgtccagccacctgtagactttgtgcaagcgatgatgtctatgatggaggcgatatcacagagagtaagtaaggttgactatcagctagatcttgtcttgaaacagacatcctccatccctatgatgcggtccgaaatccaacagctgaaaacatctgttgcagtcatggaagccaacttgggaatgatgaagattctggatcccggttgtgccaacatttcatctctgagtgatctacgggcagttgcccgatctcacccggttttagtttcaggccctggagacccctctccctatgtgacacaaggaggcgaaatggcacttaataaactttcgcaaccagtgccacatccatctgaattgattaaactcgccactgcatgcgggcctgatataggagtggaaaaggacactgtccgtgcattgatcatgtcacgcccaatgcacccgagttcttcagccaagctcctaagcaagttagatgcagccgggtcgatcgaggaaatcaggaaaatcaagcgccttgcagtgaatggctaatctagagtcgacccgggcggccgcttccctttagtgagggttaatgcttcgagcagacatgataagatacattgatgagtttggacaaaccacaactagaatgcagtgaaaaaaatgctttatttgtgaaatttgtgatgctattgctttatttgtaaccattataagctgcaataaacaagttaacaacaacaattgcattcattttatgtttcaggttcagggggagatgtgggaggttttttaaagcaagtaaaacctctacaaatgtggta

SEQ ID NO: 41 - DNA, 7989 bp, Artificial Sequence
  Artificial sequence
tcaatattggccattagccatattattcattggttatatagcataaatcaatattggctattggccattgcatacgttgtatctatatcataatatgtacatttatattggctcatgtccaatatgaccgccatgttggcattgattattgactagttattaatagtaatcaattacggggtcattagttcatagcccatatatggagttccgcgttacataacttacggtaaatggcccgcctggctgaccgcccaacgacccccgcccattgacgtcaataatgacgtatgttcccatagtaacgccaatagggactttccattgacgtcaatgggtggagtatttacggtaaactgcccacttggcagtacatcaagtgtatcatatgccaagtccgccccctattgacgtcaatgacggtaaatggcccgcctggcattatgcccagtacatgaccttacgggactttcctacttggcagtacatctacgtattagtcatcgctattaccatggtgatgcggttttggcagtacaccaatgggcgtggatagcggtttgactcacggggatttccaagtctccaccccattgacgtcaatgggagtttgttttggcaccaaaatcaacgggactttccaaaatgtcgtaacaactgcgatcgcccgccccgttgacgcaaatgggcggtaggcgtgtacggtgggaggtctatataagcagagctcgtttagtgaaccgtcagatcactagaagctttattgcggtagtttatcacagttaaattgctaacgcagtcagtgcttctgacacaacagtctcgaacttaagctgcagtgactctcttaaggtagccttgcagaagttggtcgtgaggcactgggcaggtaagtatcaaggttacaagacaggtttaaggagaccaatagaaactgggcttgtcgagacagagaagactcttgcgtttctgataggcacctattggtcttactgacatccactttgcctttctctccacaggtgtccactcccagttcaattacagctcttaaggctagagtacttaatacgactcactataggctagcctcgagaattcacgcgtaattatggcgagctccggtcctgaaagggcagagcatcagattatcctaccagagccacacctgtcttcaccattggtcaagcacaaactactctattactggaaattaactgggctaccgcttcctgatgaatgtgacttcgaccacctcattctcagccgacaatggaaaaaaatacttgaatcggcctctcctgatactgagagaatgataaaactcggaagggcagtacaccaaactcttaaccacaattccagaataaccggagtgctccaccccaggtgtttagaacaactggctaatattgaggtcccagattcaaccaacaaatttcggaagattgagaagaagatccaaattcacaacacgagatatggagaactgttcacaaggctgtgtacgcatatagagaagaaactgctggggtcatcttggtctaacaatgtcccccggtcagaggagttcagcagcattcgtacggatccggcattctggtttcactcaaaatggtccacagccaagtttgcatggctccatataaaacagatccagaggcatctgatggtggcagctaagacaaggtctgcggccaacaaattggtgatgctaacccataaggtaggccaagtctttgtcactcctgaacttgtcgttgtgacgcatacgaatgagaacaagttcacatgtcttacccaggaacttgtattgatgtatgcagatatgatggagggcagagatatggtcaacataatatcaaccacggcggtgcatctcagaagcttatcagagaaaattgatgacattttgcggttaatagacgctctggcaaaagacttgggtaatcaagtctacgatgttgtatcactaatggagggatttgcatacggagctgtccagctactcgagccgtcaggtacatttgcaggagatttcttcgcattcaacctgcaggagcttaaagacattctaattggcctcctccccaatgatatagcagaatccgtgactcatgcaatcgctactgtattctctggtttagaacagaatcaagcagctgagatgttgtgtctgttgcgtctgtggggtcacccactgcttgagtcccgtattgcagcaaaggcagtcaggagccaaatgtgcgcaccgaaaatggtagactttgatatgatccttcaggtactgtctttcttcaagggaacaatcatcaacgggtacagaaagaagaatgcaggtgtgtggccgcgagtcaaagtggatacaatatatgggaaggtcattgggcaactacatgcagattcagcagagatttcacacgatatcatgttgagagagtataagagtttatctgcacttgaatttgagccatgtatagaatatgaccctgtcaccaacctgagcatgttcctaaaagacaaggcaatcgcacaccccaacgataattggcttgcctcgtttaggcggaaccttctctccgaagaccagaagaaacatgtaaaagaagcaacttcgactaatcgcctcttgatagagtttttagagtcaaatgattttgatccatataaagagatggaatatctgacgacccttgagtaccttagagatgacaatgtggcagtatcatactcgctcaaggagaaggaagtgaaagttaatggacggatcttcgctaagctgacaaagaagttaaggaactgtcaggtgatggcggaagggatcctagccgatcagattgcacctttctttcagggaaatggagtcattcaggatagcatatccttgaccaagagtatgctagcgatgagtcaactgtcttttaacagcaataagaaacgtatcactgactgtaaagaaagagtatcttcaaaccgcaatcatgatccgaaaagcaagaaccgtcggagagttgcaaccttcataacaactgacctgcaaaagtactgtcttaattggagatatcagacaatcaaattgttcgctcatgccatcaatcagttgatgggcctacctcacttcttcgaatggattcacctaagactgatggacactacgatgttcgtaggagaccctttcaatcctccaagtgaccctactgactgtgacctctcaagagtccctaatgatgacatatatattgtcagtgccagagggggtatcgaaggattatgccagaagctatggacaatgatctcaattgctgcaatccaacttgctgcagctagatcgcattgtcgtgttgcctgtatggtacagggtgataatcaagtaatagcagtaacgagagaggtaagatcagacgactctccggagatggtgttgacacagttgcatcaagccagtgataatttcttcaaggaattaattcatgtcaatcatttgattggccataatttgaaggatcgtgaaaccatcaggtcagacacattcttcatatacagcaaacgaatcttcaaagatggagcaatcctcagtcaagtcctcaaaaattcatctaaattagtgctagtgtcaggtgatctcagtgaaaacaccgtaatgtcctgtgccaacattgcctctactgtagcacggctatgcgagaacgggcttcccaaagacttctgttactatttaaactatataatgagttgtgtgcagacatactttgactctgagttctccatcaccaacaattcgcaccccgatcttaatcagtcgtggattgaggacatctcttttgtgcactcatatgttctgactcctgcccaattagggggactgagtaaccttcaatactcaaggctctacactagaaatatcggtgacccggggactactgcttttgcagagatcaagcgactagaagcagtgggattactgagtcctaacattatgactaatatcttaactaggccgcctgggaatggagattgggccagtctgtgcaacgacccatactctttcaattttgagactgttgcaagcccaaatattgttcttaagaaacatacgcaaagagtcctatttgaaacttgttcaaatcccttattgtctggagtgcacacagaggataatgaggcagaagagaaggcattggctgaattcttgcttaatcaagaggtgattcatccccgcgttgcgcatgccatcatggaggcaagctctgtaggtaggagaaagcaaattcaagggcttgttgacacaacaaacaccgtaattaagattgcgcttactaggaggccattaggcatcaagaggctgatgcggatagtcaattattctagcatgcatgcaatgctgtttagagacgatgttttttcctccagtagatccaaccaccccttagtctcttctaatatgtgttctctgacactggcagactatgcacggaatagaagctggtcacctttgacgggaggcaggaaaatactgggtgtatctaatcctgatacgatagaactcgtagagggtgagattcttagtgtaagcggagggtgtacaagatgtgacagcggagatgaacaatttacttggttccatcttccaagcaatatagaattgaccgatgacaccagcaagaatcctccgatgagggtaccatatctcgggtcaaagacacaggagaggagagctgcctcacttgcaaaaatagctcatatgtcgccacatgtaaaggctgccctaagggcatcatccgtgttgatctgggcttatggggataatgaagtaaattggactgctgctcttacgattgcaaaatctcggtgtaatgtaaacttagagtatcttcggttactgtcccctttacccacggctgggaatcttcaacatagactagatgatggtataactcagatgacattcacccctgcatctctctacagggtgtcaccttacattcacatatccaatgattctcaaaggctgttcactgaagaaggagtcaaagaggggaatgtggtttaccaacagatcatgctcttgggtttatctctaatcgaatcgatctttccaatgacaacaaccaggacatatgatgagatcacactgcacctacatagtaaatttagttgctgtatcagagaagcacctgttgcggttcctttcgagctacttggggtggtaccggaactgaggacagtgacctcaaataagtttatgtatgatcctagccctgtatcggagggagactttgcgagacttgacttagctatcttcaagagttatgagcttaatctggagtcatatcccacgatagagctaatgaacattctttcaatatccagcgggaagttgattggccagtctgtggtttcttatgatgaagatacctccataaagaatgacgccataatagtgtatgacaatacccgaaattggatcagtgaagctcagaattcagatgtggtccgcctatttgaatatgcagcacttgaagtgctcctcgactgttcttaccaactctattacctgagagtaagaggcctagacaatattgtcttatatatgggtgatttatacaagaatatgccaggaattctactttccaacattgcagctacaatatctcatcccgtcattcattcaaggttacatgcagtgggcctggtcaaccatgacggatcacaccaacttgcagatacggattttatcgaaatgtctgcaaaactattagtatcttgcacccgacgtgtgatctccggcttatattcaggaaataagtatgatctgctgttcccatctgtcttagatgataacctgaatgagaagatgcttcagctgatatcccggttatgctgtctgtacacggtactctttgctacaacaagagaaatcccgaaaataagaggcttaactgcagaagagaaatgttcaatactcactgagtatttactgtcggatgctgtgaaaccattacttagccccgatcaagtgagctctatcatgtctcctaacataattacattcccagctaatctgtactacatgtctcggaagagcctcaatttgatcagggaaagggaggacagggatactatcctggcgttgttgttcccccaagagccattattagagttcccttctgtgcaagatattggtgctcgagtgaaagatccattcacccgacaacctgcggcatttttgcaagagttagatttgagtgctccagcaaggtatgacgcattcacacttagtcagattcatcctgaactcacatctccaaatccggaggaagactacttagtacgatacttgttcagagggatagggactgcatcttcctcttggtataaggcatctcatctcctttctgtacccgaggtaagatgtgcaagacacgggaactccttatacttagctgaagggagcggagccatcatgagtcttctcgaactgcatgtaccacatgaaactatctattacaatacgctcttttcaaatgagatgaaccccccgcaacgacatttcgggccgaccccaactcagtttttgaattcggttgtttataggaatctacaggcggaggtaacatgcaaagatggatttgtccaagagttccgtccattatggagagaaaatacagaggaaagtgacctgacctcagataaagcagtggggtatattacatctgcagtgccctacagatctgtatcattgctgcattgtgacattgaaattcctccagggtccaatcaaagcttactagatcaactagctatcaatttatctctgattgccatgcattctgtaagggagggcggggtagtaatcatcaaagtgttgtatgcaatgggatactactttcatctactcatgaacttgtttgctccgtgttccacaaaaggatatattctctctaatggttatgcatgtcgaggagatatggagtgttacctggtatttgtcatgggttacctgggcgggcctacatttgtacatgaggtggtgaggatggcaaaaactctggtgcagcggcacggtacgctcttgtctaaatcagatgagatcacactgaccaggttattcacctcacagcggcagcgtgtgacagacatcctatccagtcctttaccaagattaataaagtacttgaggaagaatattgacactgcgctgattgaagccgggggacagcccgtccgtccattctgtgcggagagtctggtgagcacgctagcgaacataactcagataacccagattatcgctagtcacattgacacagttatccggtctgtgatatatatggaagctgagggtgatctcgctgacacagtatttctatttaccccttacaatctctctactgacgggaaaaagaggacatcacttatacagtgcacgagacagatcctagaggttacaatactaggtcttagagtcgaaaatctcaataaaataggcgatataatcagcctagtgcttaaaggcatgatctcaatggaggaccttatcccactaaggacatacttgaagcatagtacctgccctaaatatttgaaggctgtcctaggtattaccaaactcaaagaaatgtttacagacacttctgtattgtacttgactcgtgctcaacaaaaattctacatgaaaactataggcaatgcagtcaaaggatattacagtaactgtgactcttaatgaagcggccgcttccctttagtgagggttaatgcttcgagcagacatgataagatacattgatgagtttggacaaaccacaactagaatgcagtgaaaaaaatgctttatttgtgaaatttgtgatgctattgctttatttgtaaccattataagctgcaataaacaagttaacaacaacaattgcattcattttatgtttcaggttcagggggagatgtgggaggttttttaaagcaagtaaaacctctacaaatgtggta

SEQ ID NO: 42 - DNA, 2655 bp, T7 bacteriophage
atgaacacgattaacatcgctaagaacgacttctctgacatcgaactggctgctatcccgttcaacactctggctgaccattacggtgagcgtttagctcgcgaacagttggcccttgagcatgagtcttacgagatgggtgaagcacgcttccgcaagatgtttgagcgtcaacttaaagctggtgaggttgcggataacgctgccgccaagcctctcatcactaccctactccctaagatgattgcacgcatcaacgactggtttgaggaagtgaaagctaagcgcggcaagcgcccgacagccttccagttcctgcaagaaatcaagccggaagccgtagcgtacatcaccattaagaccactctggcttgcctaaccagtgctgacaatacaaccgttcaggctgtagcaagcgcaatcggtcgggccattgaggacgaggctcgcttcggtcgtatccgtgaccttgaagctaagcacttcaagaaaaacgttgaggaacaactcaacaagcgcgtagggcacgtctacaagaaagcatttatgcaagttgtcgaggctgacatgctctctaagggtctactcggtggcgaggcgtggtcttcgtggcataaggaagactctattcatgtaggagtacgctgcatcgagatgctcattgagtcaaccggaatggttagcttacaccgccaaaatgctggcgtagtaggtcaagactctgagactatcgaactcgcacctgaatacgctgaggctatcgcaacccgtgcaggtgcgctggctggcatctctccgatgttccaaccttgcgtagttcctcctaagccgtggactggcattactggtggtggctattgggctaacggtcgtcgtcctctggcgctggtgcgtactcacagtaagaaagcactgatgcgctacgaagacgtttacatgcctgaggtgtacaaagcgattaacattgcgcaaaacaccgcatggaaaatcaacaagaaagtcctagcggtcgccaacgtaatcaccaagtggaagcattgtccggtcgaggacatccctgcgattgagcgtgaagaactcccgatgaaaccggaagacatcgacatgaatcctgaggctctcaccgcgtggaaacgtgctgccgctgctgtgtaccgcaaggacaaggctcgcaagtctcgccgtatcagccttgagttcatgcttgagcaagccaataagtttgctaaccataaggccatctggttcccttacaacatggactggcgcggtcgtgtttacgctgtgtcaatgttcaacccgcaaggtaacgatatgaccaaaggactgcttacgctggcgaaaggtaaaccaatcggtaaggaaggttactactggctgaaaatccacggtgcaaactgtgcgggtgtcgataaggttccgttccctgagcgcatcaagttcattgaggaaaaccacgagaacatcatggcttgcgctaagtctccactggagaacacttggtgggctgagcaagattctccgttctgcttccttgcgttctgctttgagtacgctggggtacagcaccacggcctgagctataactgctcccttccgctggcgtttgacgggtcttgctctggcatccagcacttctccgcgatgctccgagatgaggtaggtggtcgcgcggttaacttgcttcctagtgaaaccgttcaggacatctacgggattgttgctaagaaagtcaacgagattctacaagcagacgcaatcaatgggaccgataacgaagtagttaccgtgaccgatgagaacactggtgaaatctctgagaaagtcaagctgggcactaaggcactggctggtcaatggctggcttacggtgttactcgcagtgtgactaagcgttcagtcatgacgctggcttacgggtccaaagagttcggcttccgtcaacaagtgctggaagataccattcagccagctattgattccggcaagggtctgatgttcactcagccgaatcaggctgctggatacatggctaagctgatttgggaatctgtgagcgtgacggtggtagctgcggttgaagcaatgaactggcttaagtctgctgctaagctgctggctgctgaggtcaaagataagaagactggagagattcttcgcaagcgttgcgctgtgcattgggtaactcctgatggtttccctgtgtggcaggaatacaagaagcctattcagacgcgcttgaacctgatgttcctcggtcagttccgcttacagcctaccattaacaccaacaaagatagcgagattgatgcacacaaacaggagtctggtatcgctcctaactttgtacacagccaagacggtagccaccttcgtaagactgtagtgtgggcacacgagaagtacggaatcgaatcttttgcactgattcacgactccttcggtaccattccggctgacgctgcgaacctgttcaaagcagtgcgcgaaactatggttgacacatatgagtcttgtgatgtactggctgatttctacgaccagttcgctgaccagttgcacgagtctcaattggacaaaatgccagcacttccggctaaaggtaacttgaacctccgtgacatcttagagtcggacttcgcgttcgcgtaataa

SEQ ID NO: 43 - DNA, 36 bp, Artificial Sequence
  primer
aaatacgcgtaattatggcgagctccggtcctgaaa

SEQ ID NO: 44 - DNA, 35 bp, Artificial Sequence
  primer
tatggatcctatttatcatcgagctcgagatctgg

SEQ ID NO: 45 - DNA, 31 bp, Artificial Sequence
  primer
catcgtctcccatgcccgccatgaagatcga

SEQ ID NO: 46 - DNA, 26 bp, Artificial Sequence
  primer
cgaattcttacgcgaacgcgaagtcc

SEQ ID NO: 47 - DNA, 29 bp, Artificial Sequence
  primer
ccggatccatgaacacgattaacatcgct

SEQ ID NO: 48 - DNA, 23 bp, Artificial Sequence
  primer
aagaccgtgttgaggtgttatta

SEQ ID NO: 49 - DNA, 22 bp, Artificial Sequence
  primer
tccccaatgtagatactgcttc

SEQ ID NO: 50 - DNA, 20 bp, Artificial Sequence
  primer
tatccagcaaggcgtgtcta

SEQ ID NO: 51 - DNA, 21 bp, Artificial Sequence
  primer
ttgtcactgtgtctgcgtctt

SEQ ID NO: 52 - DNA, 23 bp, Artificial Sequence
  primer
cactccaattctacccgtatttt

SEQ ID NO: 53 - DNA, 25 bp, Artificial Sequence
  primer
ctaccatgatcctagtgagtgtttt

SEQ ID NO: 54 - DNA, 20 bp, Artificial Sequence
  primer
gctttggttgcttgctacaa

SEQ ID NO: 55 - DNA, 20 bp, Artificial Sequence
  primer
gaaccgtgcaatggtaagaa

SEQ ID NO: 56 - DNA, 20 bp, Artificial Sequence
  primer
ggtgttgcaactgcagctgc

SEQ ID NO: 57 - DNA, 20 bp, Artificial Sequence
  primer
cttcctcagccccactgaat

SEQ ID NO: 58 - DNA, 26 bp, Artificial Sequence
  primer
accaaacagagaatccgtgagttacg

SEQ ID NO: 59 - DNA, 26 bp, Artificial Sequence
  primer
accaaacaaagatttggtgaatgacg

SEQ ID NO: 60 - DNA, 33 bp, Artificial Sequence
  primer
ataacgccggcgcctcacatggctcgacagatc

SEQ ID NO: 61 - DNA, 39 bp, Artificial Sequence
  primer
tataggccggccacgccagcccggatcgatccttatcgg

SEQ ID NO: 62 - DNA, 26 bp, Artificial Sequence
  primer
atggtgatggtgatggtggcttcccc

SEQ ID NO: 63 - DNA, 25 bp, Artificial Sequence
  primer
ggtggcttccccttggcaccagtcc

SEQ ID NO: 64 - DNA, 22 bp, Artificial Sequence
  primer
atagcgcccagcacgaatctcc

SEQ ID NO: 65 - DNA, 20 bp, Artificial Sequence
  primer
tgccgcacgacgttcaggaa

SEQ ID NO: 66 - DNA, 20 bp, Artificial Sequence
  primer
tggtcctctctcagcaggca

SEQ ID NO: 67 - DNA, 20 bp, Artificial Sequence
  primer
agcccttgttcagctgcttg

SEQ ID NO: 68 - DNA, 20 bp, Artificial Sequence
  primer
gaaagtaaggtccaattgcc

SEQ ID NO: 69 - DNA, 20 bp, Artificial Sequence
  primer
cagagtgggcatcatcaagc

SEQ ID NO: 70 - DNA, 20 bp, Artificial Sequence
  primer
tggcgagaagggcaactacg

SEQ ID NO: 71 - DNA, 20 bp, Artificial Sequence
  primer
cagttcaaccggcggttcct

SEQ ID NO: 72 - DNA, 20 bp, Artificial Sequence
  primer
agatcgagaaccctcgggct

SEQ ID NO: 73 - DNA, 22 bp, Artificial Sequence
  primer
aaacttgtcgacgctagcgccg

SEQ ID NO: 74 - DNA, 35 bp, Artificial Sequence
  primer
ccagctcgagtcattagccatttagagcaaggcgc

SEQ ID NO: 75 - DNA, 36 bp, Artificial Sequence
  primer
ccgcatcgtctcccatggccacctttacagatgcag

SEQ ID NO: 76 - DNA, 37 bp, Artificial Sequence
  primer
ttatctcgagttttatcagtacccccagtcggtgtcg

SEQ ID NO: 77 - DNA, 30 bp, Artificial Sequence
  primer
cgcatacatgtcttccgtatttgatgagta

SEQ ID NO: 78 - DNA, 28 bp, Artificial Sequence
  primer
caaaggatattacagtaactgtgactct

SEQ ID NO: 79 - DNA, 20 bp, Artificial Sequence
  primer
actgcgctgattgaagccgg

SEQ ID NO: 80 - DNA, 20 bp, Artificial Sequence
  primer
catctgcagtgccctacaga

SEQ ID NO: 81 - DNA, 20 bp, Artificial Sequence
  primer
cattcacccgacaacctgcg

SEQ ID NO: 82 - DNA, 21 bp, Artificial Sequence
  primer
tcacaccaacttgcagatacg

SEQ ID NO: 83 - DNA, 20 bp, Artificial Sequence
  primer
accggaactgaggacagtga

SEQ ID NO: 84 - DNA, 20 bp, Artificial Sequence
  primer
acaggagaggagagctgcct

SEQ ID NO: 85 - DNA, 20 bp, Artificial Sequence
  primer
tgattcatccccgcgttgcg

SEQ ID NO: 86 - DNA, 28 bp, Artificial Sequence
  primer
gcttcccaaagacttctgttactattta

SEQ ID NO: 87 - DNA, 21 bp, Artificial Sequence
  primer
tgtgacctctcaagagtccct

SEQ ID NO: 88 - DNA, 22 bp, Artificial Sequence
  primer
ccttagagatgacaatgtggca

SEQ ID NO: 89 - DNA, 20 bp, Artificial Sequence
  primer
gcttgagtcccgtattgcag

SEQ ID NO: 90 - DNA, 22 bp, Artificial Sequence
  primer
caacaaattggtgatgctaacc

SEQ ID NO: 91 - DNA, 28 bp, Artificial Sequence
  primer
caagcacaaactactctattactggaaa

SEQ ID NO: 92 - DNA, 21 bp, Artificial Sequence
  primer
caagcagtaccaaagcagcat

SEQ ID NO: 93 - DNA, 20 bp, Artificial Sequence
  primer
attcgaatggccaagtcttc

SEQ ID NO: 94 - DNA, 23 bp, Artificial Sequence
  primer
cccattactgctacacccataat

SEQ ID NO: 95 - DNA, 24 bp, Artificial Sequence
  primer
gcaaaaaatacatggcgcttgata

SEQ ID NO: 96 - DNA, 25 bp, Artificial Sequence
  primer
caactcgatcagtaatgctttgaat

SEQ ID NO: 97 - DNA, 20 bp, Artificial Sequence
  primer
cgtaagcacaaccaggggat

SEQ ID NO: 98 - DNA, 22 bp, Artificial Sequence
  primer
agctctgatacaagccaaacaa

SEQ ID NO: 99 - DNA, 22 bp, Artificial Sequence
  primer
cccagatcatcatgacacaaaa

SEQ ID NO: 100 - DNA, 21 bp, Artificial Sequence
  primer
ttgtctaagtctgacagcgga

SEQ ID NO: 101 - DNA, 23 bp, Artificial Sequence
  primer
cagtattcatcaccacctatgga

SEQ ID NO: 102 - DNA, 20 bp, Artificial Sequence
  primer
tgatcatgtcacgcccaatg

SEQ ID NO: 103 - DNA, 22 bp, Artificial Sequence
  primer
cacaactatcagctggtgcaac

SEQ ID NO: 104 - DNA, 20 bp, Artificial Sequence
  primer
ttacagcccagggtaaacca

SEQ ID NO: 105 - DNA, 20 bp, Artificial Sequence
  primer
cccaattcctggatctgatg

SEQ ID NO: 106 - DNA, 20 bp, Artificial Sequence
  primer
gacatcagcccttgcactta

SEQ ID NO: 107 - DNA, 20 bp, Artificial Sequence
  primer
gccccagttcaacaatagga

SEQ ID NO: 108 - DNA, 22 bp, Artificial Sequence
  primer
ccctttcgtcttcaagaattct

SEQ ID NO: 109 - DNA, 20 bp, Artificial Sequence
  primer
ttgttgaactggggcgtgcc

SEQ ID NO: 110 - DNA, 20 bp, Artificial Sequence
  primer
aacgcatgagctgcttcatc

SEQ ID NO: 111 - DNA, 20 bp, Artificial Sequence
  primer
tcgttatcttgggatggccc

SEQ ID NO: 112 - DNA, 21 bp, Artificial Sequence
  primer
gggtgtggatggttgtttgtc

SEQ ID NO: 113 - DNA, 20 bp, Artificial Sequence
  primer
gatttcggaccgcatcatag

SEQ ID NO: 114 - DNA, 20 bp, Artificial Sequence
  primer
attaattacggttggccggc

SEQ ID NO: 115 - DNA, 20 bp, Artificial Sequence
  primer
ttctctggcgctttcacgtg

SEQ ID NO: 116 - DNA, 25 bp, Artificial Sequence
  primer
tagaggtaacctcgtggtcggcggt

SEQ ID NO: 117 - DNA, 21 bp, Artificial Sequence
  primer
ccccctccagatgtagtcaca

SEQ ID NO: 118 - DNA, 21 bp, Artificial Sequence
  primer
ttaggttcccgactgaaggta

SEQ ID NO: 119 - DNA, 28 bp, Artificial Sequence
  primer
ctgttgctttcctctaacttattcaaag

SEQ ID NO: 120 - DNA, 26 bp, Artificial Sequence
  primer
gctacagatatagccaaggtcactac

SEQ ID NO: 121 - DNA, 24 bp, Artificial Sequence
  primer
cgcagagtagaaaagaataccctc

SEQ ID NO: 122 - DNA, 23 bp, Artificial Sequence
  primer
ccctactgtgagaattctgcctt

SEQ ID NO: 123 - DNA, 23 bp, Artificial Sequence
  primer
gatacaatgccatctttccaact

SEQ ID NO: 124 - DNA, 25 bp, Artificial Sequence
  primer
gtgaatttggatcttcttctcaatc

SEQ ID NO: 125 - DNA, 20 bp, Artificial Sequence
  primer
gctcgagtagctggacagct

SEQ ID NO: 126 - DNA, 20 bp, Artificial Sequence
  primer
cctaaacgaggcaagccaat

SEQ ID NO: 127 - DNA, 20 bp, Artificial Sequence
  primer
tgaggtaggcccatcaactg

SEQ ID NO: 128 - DNA, 20 bp, Artificial Sequence
  primer
cagtagaggcaatgttggca

SEQ ID NO: 129 - DNA, 20 bp, Artificial Sequence
  primer
gcggggatgaatcacctctt

SEQ ID NO: 130 - DNA, 20 bp, Artificial Sequence
  primer
ccttagggcagcctttacat

SEQ ID NO: 131 - DNA, 26 bp, Artificial Sequence
  primer
tgactccagattaagctcataactct

SEQ ID NO: 132 - DNA, 21 bp, Artificial Sequence
  primer
cgggatatcagctgaagcatc

SEQ ID NO: 133 - DNA, 22 bp, Artificial Sequence
  primer
ccgtgtcttgcacatcttacct

SEQ ID NO: 134 - DNA, 22 bp, Artificial Sequence
  primer
aacactccatatctcctcgaca

SEQ ID NO: 135 - DNA, 21 bp, Artificial Sequence
  primer
atggagatcatgcctttaagc

SEQ ID NO: 136 - DNA, 24 bp, Artificial Sequence
  primer
gtgataaactaccgcattaaagct